European Patent Specification EP 3 368 695 B1, published June 25, 2025. Title: METHOD FOR PRODUCING ALDEHYDE. Applicant: Ajinomoto Co., Inc. The sequence listing filed with the application follows.

SEQUENCE LISTING (102 sequences)

SEQ ID NO: 1 - DNA, 68 bp, Artificial Sequence
  primer
caggcagatcgttctctgccctcatattggcccagcaaagggagcaagtatctagacgctcaagttag

SEQ ID NO: 2 - DNA, 76 bp, Artificial Sequence
  primer
cttaagtctggacgaaatgcccgaaaacgaaagtttgaggcgtaaaaagcagatcttgaagcctgcttttttatac

SEQ ID NO: 3 - DNA, 20 bp, Artificial Sequence
  primer
agaaataggcaagacattgg

SEQ ID NO: 4 - DNA, 20 bp, Artificial Sequence
  primer
ggattagccatacgttcctc

SEQ ID NO: 5 - DNA, 51 bp, Artificial Sequence
  primer
ccatgattacgaattccccctgttgacaattaatcatcggctcgtataatg

SEQ ID NO: 6 - DNA, 38 bp, Artificial Sequence
  primer
cgaccatattcgagatcctgtgtgaaattgttatccgc

SEQ ID NO: 7 - DNA, 20 bp, Artificial Sequence
  primer
tctcgaatatggtcgatatg

SEQ ID NO: 8 - DNA, 35 bp, Artificial Sequence
  primer
atgcctgcaggtcgaccgcatatccggttgtcagg

SEQ ID NO: 9 - DNA, 35 bp, Artificial Sequence
  primer
ccaagcttgcatgccagatcgtttagatccgaagg

SEQ ID NO: 10 - DNA, 20 bp, Artificial Sequence
  primer
tgtatgtcctcctggacttc

SEQ ID NO: 11 - DNA, 35 bp, Artificial Sequence
  primer
ccaggaggacatacaatggcaactgacagcaggag

SEQ ID NO: 12 - DNA, 33 bp, Artificial Sequence
  primer
gtatgtcctcctttataacagacctaaatgacg

SEQ ID NO: 13 - DNA, 36 bp, Artificial Sequence
  primer
aaaggaggacatacaatggtcgatatgaaaactacg

SEQ ID NO: 14 - DNA, 35 bp, Artificial Sequence
  primer
cggtacccggggatcccgcatatccggttgtcagg

SEQ ID NO: 15 - DNA, 35 bp, Artificial Sequence
  primer
cggtacccggggatccttacttccgcgtatccaac

SEQ ID NO: 16 - DNA, 41 bp, Artificial Sequence
  primer
ctaggaatcgcggccggtgaactcctaaagaactatataac

SEQ ID NO: 17 - DNA, 20 bp, Artificial Sequence
  primer
ggccgcgattcctagcatgc

SEQ ID NO: 18 - DNA, 35 bp, Artificial Sequence
  primer
ccaagcttgcatgccagtcatcatcaacggtgccg

SEQ ID NO: 19 - DNA, 21 bp, Artificial Sequence
  primer
atctccgcagaagacgtactg

SEQ ID NO: 20 - DNA, 20 bp, Artificial Sequence
  primer
tccgatcatgtatgacctcc

SEQ ID NO: 21 - DNA, 36 bp, Artificial Sequence
  primer
cggtacccggggatcggcatagtgcttccaacgctc

SEQ ID NO: 22 - DNA, 36 bp, Artificial Sequence
  primer
tagctccactcaagattcctcgatattacctacagg

SEQ ID NO: 23 - DNA, 20 bp, Artificial Sequence
  primer
tcttgagtggagctagggcc

SEQ ID NO: 24 - DNA, 37 bp, Artificial Sequence
  primer
ccaagcttgcatgcccatatagagcccaggagctctc

SEQ ID NO: 25 - DNA, 23 bp, Artificial Sequence
  primer
cgccgcaaagtccaaatagaaag

SEQ ID NO: 26 - DNA, 20 bp, Artificial Sequence
  primer
ggattcttcctgaactcagc

SEQ ID NO: 27 - DNA, 36 bp, Artificial Sequence
  primer
cggtacccggggatcgggctcgtcctgaaattgcac

SEQ ID NO: 28 - DNA, 35 bp, Artificial Sequence
  primer
tccgtcgtgagccatgttgtgcccacgagactacc

SEQ ID NO: 29 - DNA, 20 bp, Artificial Sequence
  primer
atggctcacgacggattgcg

SEQ ID NO: 30 - DNA, 36 bp, Artificial Sequence
  primer
ccaagcttgcatgcccggttgcagccttcataaacg

SEQ ID NO: 31 - DNA, 21 bp, Artificial Sequence
  primer
agaccaatgagtacccaaccg

SEQ ID NO: 32 - DNA, 20 bp, Artificial Sequence
  primer
tcagcgtctggctcagctac

SEQ ID NO: 33 - DNA, 36 bp, Artificial Sequence
  primer
cggtacccggggatcaaccccagctcaaataacacc

SEQ ID NO: 34 - DNA, 37 bp, Artificial Sequence
  primer
tttcaacacaatccgtccttctcgcttggattacttg

SEQ ID NO: 35 - DNA, 23 bp, Artificial Sequence
  primer
cggattgtgttgaaattgctctg

SEQ ID NO: 36 - DNA, 35 bp, Artificial Sequence
  primer
ccaagcttgcatgcctcaccacgggaatcttcagg

SEQ ID NO: 37 - DNA, 20 bp, Artificial Sequence
  primer
ccggactggggtgtgttttg

SEQ ID NO: 38 - DNA, 20 bp, Artificial Sequence
  primer
cccggaaaatacggtatagc

SEQ ID NO: 39 - DNA, 47 bp, Artificial Sequence
  primer
ccaagcttgcatgccaggaggattataatgcgcctgcgtgtctcgag

SEQ ID NO: 40 - DNA, 34 bp, Artificial Sequence
  primer
cggtacccggggatccaactacgcggcgacgtac

SEQ ID NO: 41 - DNA, 2304 bp, Homo sapiens
cggcctgcgtccgccaccggaagcgccctcctaatccccgcagcgccaccgccattgccgccatcgtcgtggggcttctggggcagctagggctgcccgccgcgctgcctgcgccggaccggggcgggtccagtcccgggcgggccgtcgcgggagagaaataacatctgctttgctgccgagctcagaggagaccccagacccctcccgcagccagagggctggagcctgctcagaggtgctttgaagatgccggaggccccgcctctgctgttggcagctgtgttgctgggcctggtgctgctggtggtgctgctgctgcttctgaggcactggggctggggcctgtgccttatcggctggaacgagttcatcctgcagcccatccacaacctgctcatgggtgacaccaaggagcagcgcatcctgaaccacgtgctgcagcatgcggagcccgggaacgcacagagcgtgctggaggccattgacacctactgcgagcagaaggagtgggccatgaacgtgggcgacaagaaaggcaagatcgtggacgccgtgattcaggagcaccagccctccgtgctgctggagctgggggcctactgtggctactcagctgtgcgcatggcccgcctgctgtcaccaggggcgaggctcatcaccatcgagatcaaccccgactgtgccgccatcacccagcggatggtggatttcgctggcgtgaaggacaaggtcacccttgtggttggagcgtcccaggacatcatcccccagctgaagaagaagtatgatgtggacacactggacatggtcttcctcgaccactggaaggaccggtacctgccggacacgcttctcttggaggaatgtggcctgctgcggaaggggacagtgctactggctgacaacgtgatctgcccaggtgcgccagacttcctagcacacgtgcgcgggagcagctgctttgagtgcacacactaccaatcgttcctggaatacagggaggtggtggacggcctggagaaggccatctacaagggcccaggcagcgaagcagggccctgactgcccccccggcccccctctcgggctctctcacccagcctggtactgaaggtgccagacgtgctcctgctgaccttctgcggctccgggctgtgtcctaaatgcaaagcacacctcggccgaggcctgcgccctgacatgctaacctctctgaactgcaacactggattgttcttttttaagactcaatcatgacttctttactaacactggctagctatattatcttatatactaatatcatgttttaaaaatataaaatagaaattaagaatctaaatatttagatataactcgacttagtacatccttctcaactgccattcccctgctgcccttgacttgggcaccaaacattcaaagctccccttgacggacgctaacgctaagggcggggcccctagctggctgggttctgggtggcacgcctggcccactggcctcccagccacagtggtgcagaggtcagccctcctgcagctaggccaggggcacctgttagccccatggggacgactgccggcctgggaaacgaagaggagtcagccagcattcacacctttctgaccaagcaggcgctggggacaggtggaccccgcagcagcaccagcccctctgggccccatgtggcacagagtggaagcatctccttccctactccccactgggccttgcttacagaagaggcaatggctcagaccagctcccgcatccctgtagttgcctccctggcccatgagtgaggatgcagtgctggtttctgcccacctacacctagagctgtccccatctcctccaaggggtcagactgctagccacctcagaggctccaagggcccagttcccaggcccaggacaggaatcaaccctgtgctagctgagttcacctgcaccgagaccagcccctagccaagattctactcctgggctcaaggcctggctagcccccagccagcccactcctatggatagacagaccagtgagcccaagtggacaagtttggggccacccagggaccagaaacagagcctctgcaggacacagcagatgggcacctgggaccacctccacccagggccctgccccagacgcgcagaggcccgacacaagggagaagccagccacttgtgccagacctgagtggcagaaagcaaaaagttcctttgctgctttaatttttaaattttcttacaaaaatttaggtgtttaccaatagtcttattttggcttatttttaa

SEQ ID NO: 42 - DNA, 2262 bp, Homo sapiens
ctcccacgggaggagcaagaacacagaacagagggggcaagacagctccaccaggagtcaggagtgaatcccctctgggaacgaggcactaggaagaagaacttccagcccaggagaaataacatctgctttgctgccgagctcagaggagaccccagacccctcccgcagccagagggctggagcctgctcagaggtgctttgaagatgccggaggccccgcctctgctgttggcagctgtgttgctgggcctggtgctgctggtggtgctgctgctgcttctgaggcactggggctggggcctgtgccttatcggctggaacgagttcatcctgcagcccatccacaacctgctcatgggtgacaccaaggagcagcgcatcctgaaccacgtgctgcagcatgcggagcccgggaacgcacagagcgtgctggaggccattgacacctactgcgagcagaaggagtgggccatgaacgtgggcgacaagaaaggcaagatcgtggacgccgtgattcaggagcaccagccctccgtgctgctggagctgggggcctactgtggctactcagctgtgcgcatggcccgcctgctgtcaccaggggcgaggctcatcaccatcgagatcaaccccgactgtgccgccatcacccagcggatggtggatttcgctggcgtgaaggacaaggtcacccttgtggttggagcgtcccaggacatcatcccccagctgaagaagaagtatgatgtggacacactggacatggtcttcctcgaccactggaaggaccggtacctgccggacacgcttctcttggaggaatgtggcctgctgcggaaggggacagtgctactggctgacaacgtgatctgcccaggtgcgccagacttcctagcacacgtgcgcgggagcagctgctttgagtgcacacactaccaatcgttcctggaatacagggaggtggtggacggcctggagaaggccatctacaagggcccaggcagcgaagcagggccctgactgcccccccggcccccctctcgggctctctcacccagcctggtactgaaggtgccagacgtgctcctgctgaccttctgcggctccgggctgtgtcctaaatgcaaagcacacctcggccgaggcctgcgccctgacatgctaacctctctgaactgcaacactggattgttcttttttaagactcaatcatgacttctttactaacactggctagctatattatcttatatactaatatcatgttttaaaaatataaaatagaaattaagaatctaaatatttagatataactcgacttagtacatccttctcaactgccattcccctgctgcccttgacttgggcaccaaacattcaaagctccccttgacggacgctaacgctaagggcggggcccctagctggctgggttctgggtggcacgcctggcccactggcctcccagccacagtggtgcagaggtcagccctcctgcagctaggccaggggcacctgttagccccatggggacgactgccggcctgggaaacgaagaggagtcagccagcattcacacctttctgaccaagcaggcgctggggacaggtggaccccgcagcagcaccagcccctctgggccccatgtggcacagagtggaagcatctccttccctactccccactgggccttgcttacagaagaggcaatggctcagaccagctcccgcatccctgtagttgcctccctggcccatgagtgaggatgcagtgctggtttctgcccacctacacctagagctgtccccatctcctccaaggggtcagactgctagccacctcagaggctccaagggcccagttcccaggcccaggacaggaatcaaccctgtgctagctgagttcacctgcaccgagaccagcccctagccaagattctactcctgggctcaaggcctggctagcccccagccagcccactcctatggatagacagaccagtgagcccaagtggacaagtttggggccacccagggaccagaaacagagcctctgcaggacacagcagatgggcacctgggaccacctccacccagggccctgccccagacgcgcagaggcccgacacaagggagaagccagccacttgtgccagacctgagtggcagaaagcaaaaagttcctttgctgctttaatttttaaattttcttacaaaaatttaggtgtttaccaatagtcttattttggcttatttttaa

SEQ ID NO: 43 - DNA, 2279 bp, Homo sapiens
tggagataacacggatcgctgtgtacactgtgtgctccggttgttgcatccgagggttgatcggatggtggttcccatccagatccaagtcctggcccctgatcacagagaaacacagctggacattaaagtgaaataacatctgctttgctgccgagctcagaggagaccccagacccctcccgcagccagagggctggagcctgctcagaggtgctttgaagatgccggaggccccgcctctgctgttggcagctgtgttgctgggcctggtgctgctggtggtgctgctgctgcttctgaggcactggggctggggcctgtgccttatcggctggaacgagttcatcctgcagcccatccacaacctgctcatgggtgacaccaaggagcagcgcatcctgaaccacgtgctgcagcatgcggagcccgggaacgcacagagcgtgctggaggccattgacacctactgcgagcagaaggagtgggccatgaacgtgggcgacaagaaaggcaagatcgtggacgccgtgattcaggagcaccagccctccgtgctgctggagctgggggcctactgtggctactcagctgtgcgcatggcccgcctgctgtcaccaggggcgaggctcatcaccatcgagatcaaccccgactgtgccgccatcacccagcggatggtggatttcgctggcgtgaaggacaaggtcacccttgtggttggagcgtcccaggacatcatcccccagctgaagaagaagtatgatgtggacacactggacatggtcttcctcgaccactggaaggaccggtacctgccggacacgcttctcttggaggaatgtggcctgctgcggaaggggacagtgctactggctgacaacgtgatctgcccaggtgcgccagacttcctagcacacgtgcgcgggagcagctgctttgagtgcacacactaccaatcgttcctggaatacagggaggtggtggacggcctggagaaggccatctacaagggcccaggcagcgaagcagggccctgactgcccccccggcccccctctcgggctctctcacccagcctggtactgaaggtgccagacgtgctcctgctgaccttctgcggctccgggctgtgtcctaaatgcaaagcacacctcggccgaggcctgcgccctgacatgctaacctctctgaactgcaacactggattgttcttttttaagactcaatcatgacttctttactaacactggctagctatattatcttatatactaatatcatgttttaaaaatataaaatagaaattaagaatctaaatatttagatataactcgacttagtacatccttctcaactgccattcccctgctgcccttgacttgggcaccaaacattcaaagctccccttgacggacgctaacgctaagggcggggcccctagctggctgggttctgggtggcacgcctggcccactggcctcccagccacagtggtgcagaggtcagccctcctgcagctaggccaggggcacctgttagccccatggggacgactgccggcctgggaaacgaagaggagtcagccagcattcacacctttctgaccaagcaggcgctggggacaggtggaccccgcagcagcaccagcccctctgggccccatgtggcacagagtggaagcatctccttccctactccccactgggccttgcttacagaagaggcaatggctcagaccagctcccgcatccctgtagttgcctccctggcccatgagtgaggatgcagtgctggtttctgcccacctacacctagagctgtccccatctcctccaaggggtcagactgctagccacctcagaggctccaagggcccagttcccaggcccaggacaggaatcaaccctgtgctagctgagttcacctgcaccgagaccagcccctagccaagattctactcctgggctcaaggcctggctagcccccagccagcccactcctatggatagacagaccagtgagcccaagtggacaagtttggggccacccagggaccagaaacagagcctctgcaggacacagcagatgggcacctgggaccacctccacccagggccctgccccagacgcgcagaggcccgacacaagggagaagccagccacttgtgccagacctgagtggcagaaagcaaaaagttcctttgctgctttaatttttaaattttcttacaaaaatttaggtgtttaccaatagtcttattttggcttatttttaa

SEQ ID NO: 44 - DNA, 2035 bp, Homo sapiens
gctgttggcagctgtgttgctgggcctggtgctgctggtggtgctgctgctgcttctgaggcactggggctggggcctgtgccttatcggctggaacgagttcatcctgcagcccatccacaacctgctcatgggtgacaccaaggagcagcgcatcctgaaccacgtgctgcagcatgcggagcccgggaacgcacagagcgtgctggaggccattgacacctactgcgagcagaaggagtgggccatgaacgtgggcgacaagaaaggcaagatcgtggacgccgtgattcaggagcaccagccctccgtgctgctggagctgggggcctactgtggctactcagctgtgcgcatggcccgcctgctgtcaccaggggcgaggctcatcaccatcgagatcaaccccgactgtgccgccatcacccagcggatggtggatttcgctggcgtgaaggacaaggtcacccttgtggttggagcgtcccaggacatcatcccccagctgaagaagaagtatgatgtggacacactggacatggtcttcctcgaccactggaaggaccggtacctgccggacacgcttctcttggaggaatgtggcctgctgcggaaggggacagtgctactggctgacaacgtgatctgcccaggtgcgccagacttcctagcacacgtgcgcgggagcagctgctttgagtgcacacactaccaatcgttcctggaatacagggaggtggtggacggcctggagaaggccatctacaagggcccaggcagcgaagcagggccctgactgcccccccggcccccctctcgggctctctcacccagcctggtactgaaggtgccagacgtgctcctgctgaccttctgcggctccgggctgtgtcctaaatgcaaagcacacctcggccgaggcctgcgccctgacatgctaacctctctgaactgcaacactggattgttcttttttaagactcaatcatgacttctttactaacactggctagctatattatcttatatactaatatcatgttttaaaaatataaaatagaaattaagaatctaaatatttagatataactcgacttagtacatccttctcaactgccattcccctgctgcccttgacttgggcaccaaacattcaaagctccccttgacggacgctaacgctaagggcggggcccctagctggctgggttctgggtggcacgcctggcccactggcctcccagccacagtggtgcagaggtcagccctcctgcagctaggccaggggcacctgttagccccatggggacgactgccggcctgggaaacgaagaggagtcagccagcattcacacctttctgaccaagcaggcgctggggacaggtggaccccgcagcagcaccagcccctctgggccccatgtggcacagagtggaagcatctccttccctactccccactgggccttgcttacagaagaggcaatggctcagaccagctcccgcatccctgtagttgcctccctggcccatgagtgaggatgcagtgctggtttctgcccacctacacctagagctgtccccatctcctccaaggggtcagactgctagccacctcagaggctccaagggcccagttcccaggcccaggacaggaatcaaccctgtgctagctgagttcacctgcaccgagaccagcccctagccaagattctactcctgggctcaaggcctggctagcccccagccagcccactcctatggatagacagaccagtgagcccaagtggacaagtttggggccacccagggaccagaaacagagcctctgcaggacacagcagatgggcacctgggaccacctccacccagggccctgccccagacgcgcagaggcccgacacaagggagaagccagccacttgtgccagacctgagtggcagaaagcaaaaagttcctttgctgctttaatttttaaattttcttacaaaaatttaggtgtttaccaatagtcttattttggcttatttttaa

SEQ ID NO: 45 - protein, 271 aa, Homo sapiens
MPEAPPLLLAAVLLGLVLLVVLLLLLRHWGWGLCLIGWNEFILQPIHNLLMGDTKEQRILNHVLQHAEPGNAQSVLEAIDTYCEQKEWAMNVGDKKGKIVDAVIQEHQPSVLLELGAYCGYSAVRMARLLSPGARLITIEINPDCAAITQRMVDFAGVKDKVTLVVGASQDIIPQLKKKYDVDTLDMVFLDHWKDRYLPDTLLLEECGLLRKGTVLLADNVICPGAPDFLAHVRGSSCFECTHYQSFLEYREVVDGLEKAIYKGPGSEAGP

SEQ ID NO: 46 - protein, 221 aa, Homo sapiens
MGDTKEQRILNHVLQHAEPGNAQSVLEAIDTYCEQKEWAMNVGDKKGKIVDAVIQEHQPSVLLELGAYCGYSAVRMARLLSPGARLITIEINPDCAAITQRMVDFAGVKDKVTLVVGASQDIIPQLKKKYDVDTLDMVFLDHWKDRYLPDTLLLEECGLLRKGTVLLADNVICPGAPDFLAHVRGSSCFECTHYQSFLEYREVVDGLEKAIYKGPGSEAGP

SEQ ID NO: 47 - DNA, 3501 bp, Nocardia brasiliensis
atggcgactgattcgcgaagcgatcggctacggcgtcgaattgcacagttgttcgccgaggacgagcaggtgaaagccgcggtgccggaccaggaggtggtcgaggcgatccgggcgcccggcctgcgcctggcacagatcatggccaccgtgatggagcgctatgcggaccgccccgcggtgggacagcgggcgagcgagccggtcaccgagagcggtcgcaccaccttccggctgctcccggaattcgagaccctgacctaccgcgagctgtgggcgcgcgtccgcgcggtggccgccgcgtggcacggagatgccgaaaggcctttgcgggccggggatttcgttgctctgctgggtttcgccggcatcgattacggcaccctcgatctcgcgaacatccatctcggcctcgtcacggtgccgctgcaatccggcgccacggccccgcaactcgccgcgatcctggccgagaccacgccccgggtgctggccgcgacacccgaccatctcgatatcgccgtcgaattgctgaccgggggagcctcgccggaacggctggtggtattcgactaccgccccgcggacgacgatcaccgggcggcgctcgagtccgcgcgcagacggttgagcgacgcgggcagtgcggtggtggtcgagacgctcgacgcggtccgcgcccgcggcagcgaattgccggccgcgccgctgttcgttcccgccgcggacgaggacccgctggctctgctcatctacacctccggcagcaccggcacgcctaagggcgccatgtacaccgaaagactgaaccgcacgacgtggctgagcggggcgaaaggcgtcggcctcacgctcggctacatgccgatgagtcatattgccgggcgggcctcgttcgccggtgtgctggcccgcggcggcacggtctacttcaccgcccgcagcgatatgtcgacgctgttcgaagatctggccctggtgcggccgaccgagatgttcttcgtcccgcgcgtgtgcgacatgatcttccagcgctatcaggccgaactgtcgcggcgcgcgcccgccgcggccgcgagcccggaactcgagcaggaactgaagaccgaactgcgcttgtccgcggtcggggaccgcttactcggggcgatcgcgggcagcgcgccgctgtcggccgagatgcgggagttcatggagtcgctgctggatctggaactgcacgacggctacggctcgaccgaggcgggtatcggcgtactgcaagacaatatcgtccagcgtccgccggtcatcgattacaagctcgtcgacgtgccggaattgggctacttccggacggaccagccgcatccccgcggtgagttgctgttgaaaaccgaagggatgattccgggctacttccggcggcccgaggtgaccgcggagatcttcgacgaggacggtttctacaggaccggtgacatcgtcgccgaactcgaaccggatcggctgatctacctggaccgccgcaacaatgtgctgaaactggcccagggcgagttcgtcacggtcgcccatctggaagcggtgttcgcgaccagtccgctgatccggcagatctacatctacggcaacagcgagcgctcgttcctgctggcggtgatcgtgcccaccgcggacgcgctggccgacggtgtcaccgacgcgctgaacacggcgctgaccgaatccttgcgacagctcgcgaaagaagccgggctgcaatcctatgagctgccgcgcgagttcctggtcgaaaccgaaccgttcaccgtcgagaacggtctgctctccggtatcgcgaaactgttgcggcccaagctcaaggagcactacggcgagcgactcgagcagctgtaccgcgatatcgaggcgaaccgcaacgacgagctgatcgagctgcggcgcaccgcggccgagctgccggtgctcgaaaccgtcacgcgggctgcacgttcgatgctcggactggccgcgtcggagttgcggccggacgcgcatttcaccgatctcggcggtgattcactgtccgcgctgtcgttttcgaccctgctgcaggacatgctcgaggtcgaggtcccggtcggtgtcatcgtgagccccgccaactcgctcgccgatctggcgaaatacatcgaggccgaacggcattcgggggtgcggcggccgagcctgatctcggtgcacggtcccggcaccgagatccgtgccgccgatctcaccctggacaagttcatcgacgagcgcaccctcgctgccgcgaaagcggttccggccgcgccggcccaggcgcagaccgtcctgctcaccggggcgaacggctatctcggccgcttcctgtgcctggaatggctgcagcgactggaccagaccggcggcacgctggtctgcatcgtgcgcggtaccgacgcggccgccgcgcggaagcgcctggatgcggtgttcgacagcggtgatccggagctgctcgaccactaccggaagctggccgccgagcacctcgaggtgctcgcgggcgatatcggcgacccgaatctcggcctggacgaagcgacttggcagcggctcgccgcgaccgtcgacctgatcgtgcaccccgccgccctcgtcaaccatgtgctgccgtacagccagctgttcgggccgaatgtggtcggcaccgccgagatcatccggctggccatcaccgagcgccgtaagcccgtgacgtacctgtcgacggtcgcggtggccgcacaggtcgatcccgccggcttcgacgaggagcgcgatatccgggagatgagcgcggtgcgctccatcgacgccgggtacgcgaacggttacggcaacagcaagtgggccggcgaggtgctgctgcgcgaggcccatgatctgtgcgggctgccggtcgccgtgttccgctcggacatgatcctggcgcacagcaaatacgtcggtcagctcaacgtccccgatgtgttcacccggctcatcctgagcctggcgctcaccggcatcgcaccgtattcgttctacgggacggacagcgccgggcagcgcaggcgggcccactacgacggtctgcccgccgatttcgtcgccgaggcgatcaccaccctcggcgcgcgagccgagtcggggttccatacctacgacgtgtggaacccgtacgacgacggcatctcgctggacgaattcgtcgactggctcggcgatttcggcgtgccgatccagcggatcgacgactacgacgaatggttccggcgtttcgagaccgcgatccgcgcgctgcccgaaaagcagcgcgatgcttcgctgctaccgctgctggacgcacaccggcggccactgcgcgcggtgcgcggttcgctgttgcccgccaagaacttccaggcggcggtgcagtccgcgcggatcggccccgatcaggacatcccgcatctttccccgcagttgatcgacaagtacgtcaccgacctgcgccacctcggcctgctctga

SEQ ID NO: 48 - protein, 1166 aa, Nocardia brasiliensis
MATDSRSDRLRRRIAQLFAEDEQVKAAVPDQEVVEAIRAPGLRLAQIMATVMERYADRPAVGQRASEPVTESGRTTFRLLPEFETLTYRELWARVRAVAAAWHGDAERPLRAGDFVALLGFAGIDYGTLDLANIHLGLVTVPLQSGATAPQLAAILAETTPRVLAATPDHLDIAVELLTGGASPERLVVFDYRPADDDHRAALESARRRLSDAGSAVVVETLDAVRARGSELPAAPLFVPAADEDPLALLIYTSGSTGTPKGAMYTERLNRTTWLSGAKGVGLTLGYMPMSHIAGRASFAGVLARGGTVYFTARSDMSTLFEDLALVRPTEMFFVPRVCDMIFQRYQAELSRRAPAAAASPELEQELKTELRLSAVGDRLLGAIAGSAPLSAEMREFMESLLDLELHDGYGSTEAGIGVLQDNIVQRPPVIDYKLVDVPELGYFRTDQPHPRGELLLKTEGMIPGYFRRPEVTAEIFDEDGFYRTGDIVAELEPDRLIYLDRRNNVLKLAQGEFVTVAHLEAVFATSPLIRQIYIYGNSERSFLLAVIVPTADALADGVTDALNTALTESLRQLAKEAGLQSYELPREFLVETEPFTVENGLLSGIAKLLRPKLKEHYGERLEQLYRDIEANRNDELIELRRTAAELPVLETVTRAARSMLGLAASELRPDAHFTDLGGDSLSALSFSTLLQDMLEVEVPVGVIVSPANSLADLAKYIEAERHSGVRRPSLISVHGPGTEIRAADLTLDKFIDERTLAAAKAVPAAPAQAQTVLLTGANGYLGRFLCLEWLQRLDQTGGTLVCIVRGTDAAAARKRLDAVFDSGDPELLDHYRKLAAEHLEVLAGDIGDPNLGLDEATWQRLAATVDLIVHPAALVNHVLPYSQLFGPNVVGTAEIIRLAITERRKPVTYLSTVAVAAQVDPAGFDEERDIREMSAVRSIDAGYANGYGNSKWAGEVLLREAHDLCGLPVAVFRSDMILAHSKYVGQLNVPDVFTRLILSLALTGIAPYSFYGTDSAGQRRRAHYDGLPADFVAEAITTLGARAESGFHTYDVWNPYDDGISLDEFVDWLGDFGVPIQRIDDYDEWFRRFETAIRALPEKQRDASLLPLLDAHRRPLRAVRGSLLPAKNFQAAVQSARIGPDQDIPHLSPQLIDKYVTDLRHLGLL

SEQ ID NO: 49 - DNA, 621 bp, Escherichia coli
atgaaaactacgcatacctccctcccctttgccggacatacgctgcattttgttgagttcgatccggcgaatttttgtgagcaggatttactctggctgccgcactacgcacaactgcaacacgctggacgtaaacgtaaaacagagcatttagccggacggatcgctgctgtttatgctttgcgggaatatggctataaatgtgtgcccgcaatcggcgagctacgccaacctgtctggcctgcggaggtatacggcagtattagccactgtgggactacggcattagccgtggtatctcgtcaaccgattggcattgatatagaagaaattttttctgtacaaaccgcaagagaattgacagacaacattattacaccagcggaacacgagcgactcgcagactgcggtttagccttttctctggcgctgacactggcattttccgccaaagagagcgcatttaaggcaagtgagatccaaactgatgcaggttttctggactatcagataattagctggaataaacagcaggtcatcattcatcgtgagaatgagatgtttgctgtgcactggcagataaaagaaaagatagtcataacgctgtgccaacacgattaa

SEQ ID NO: 50 - protein, 206 aa, Escherichia coli
MKTTHTSLPFAGHTLHFVEFDPANFCEQDLLWLPHYAQLQHAGRKRKTEHLAGRIAAVYALREYGYKCVPAIGELRQPVWPAEVYGSISHCGTTALAVVSRQPIGIDIEEIFSVQTARELTDNIITPAEHERLADCGLAFSLALTLAFSAKESAFKASEIQTDAGFLDYQIISWNKQQVIIHRENEMFAVHWQIKEKIVITLCQHD

SEQ ID NO: 51 - DNA, 654 bp, Corynebacterium glutamicum
atgctggatgagtctttgtttccaaattcggcaaagttttctttcattaaaactggcgatgctgttaatttagaccatttccatcagttgcatccgttggaaaaggcactggtagcgcactcggttgatattagaaaagcagagtttggagatgccaggtggtgtgcacatcaggcactccaagctttgggacgagatagcggtgatcccattttgcgtggggaacgaggaatgccattgtggccttcttcggtgtctggttcattgacccacactgacggattccgagctgctgttgtggcgccacgattgttggtgcgttctatgggattggatgccgaacctgcggagccgttgcccaaggatgttttgggttcaatcgctcgggtgggggagattcctcaacttaagcgcttggaggaacaaggtgtgcactgcgcggatcgcctgctgttttgtgccaaggaagcaacatacaaagcgtggttcccgctgacgcataggtggcttggttttgaacaagctgagatcgacttgcgtgatgatggcacttttgtgtcctatttgctggttcgaccaactccagtgccgtttatttcaggtaaatgggtactgcgtgatggttatgtcatagctgcgactgcagtgacttga

SEQ ID NO: 52 - protein, 217 aa, Corynebacterium glutamicum
MLDESLFPNSAKFSFIKTGDAVNLDHFHQLHPLEKALVAHSVDIRKAEFGDARWCAHQALQALGRDSGDPILRGERGMPLWPSSVSGSLTHTDGFRAAVVAPRLLVRSMGLDAEPAEPLPKDVLGSIARVGEIPQLKRLEEQGVHCADRLLFCAKEATYKAWFPLTHRWLGFEQAEIDLRDDGTFVSYLLVRPTPVPFISGKWVLRDGYVIAATAVT

SEQ ID NO: 53 - DNA, 1428 bp, Corynebacterium glutamicum
atgcgcctgcgtgtctcgagtagtctcctccccttcctcgtccccaacctcgaccattacggtcgccctctcctaaaggagcctggcatggatatccgccaaacaattaacgacacagcaatgtcgagatatcagtggttcattgtatttatcgcagtgctgctcaacgcactggacggctttgatgtcctcgccatgtcttttactgcgaatgcagtgaccgaagaatttggactgagtggcagccagcttggtgtgctgctgagttccgcgctgttcggcatgaccgctggatctttgctgttcggtccgatcggtgaccgtttcggccgtaagaatgccctgatgatcgcgctgctgttcaacgtggtgggattggtattgtccgccaccgcgcagtccgcaggccagttgggcgtgtggcgtttgatcactggtatcggcatcggcggaatcctcgcctgcatcacagtggtgatcagtgagttctccaacaacaaaaaccgcggcatggccatgtccatctacgctgctggttacggcatcggcgcgtccttgggcggattcggcgcagcgcagctcatcccaacatttggatggcgctccgtgttcgcagccggtgcgatcgcaactggtatcgccaccatcgctactttcttcttcctgccagaatccgttgattggctgagcactcgccgccctgcgggcgctcgcgacaagatcaattacattgcgcgccgcctgggcaaagtcggtacctttgagcttccaggcgaacaaagcttgtcgacgaaaaaagccggtctccaatcgtatgcagtgctcgttaacaaagagaaccgtggaaccagcatcaagctgtgggttgcgttcggcatcgtgatgttcggcttctacttcgccaacacttggaccccgaagctgctcgtggaaaccggaatgtcagaacagcagggcatcatcggtggtttgatgttgtccatgggtggagcattcggttccctgctctacggtttcctcaccaccaagttcagctcccgaaacacactgatgaccttcatggtgctgtccggcctgacgctgatcctgttcatttcctccacctctgttccatccatcgcgtttgccagcggcgttgtcgtgggcatgctgatcaatggttgtgtggctggtctgtacaccctgtccccacagctgtactccgctgaagtacgcaccactggtgtgggcgctgcgattggtatgggtcgtgtcggtgcgatttccgcgccactgctggtgggtagcctgctggattctggctggtccccaacgcagctgtatgttggtgtggcagtgattgttattgccggtgcaaccgcattgattgggatgcgcactcaggcagtagccgtcgaaaagcagcctgaagccctagcgaccaaatag

SEQ ID NO: 54 - protein, 475 aa, Corynebacterium glutamicum
MRLRVSSSLLPFLVPNLDHYGRPLLKEPGMDIRQTINDTAMSRYQWFIVFIAVLLNALDGFDVLAMSFTANAVTEEFGLSGSQLGVLLSSALFGMTAGSLLFGPIGDRFGRKNALMIALLFNVVGLVLSATAQSAGQLGVWRLITGIGIGGILACITVVISEFSNNKNRGMAMSIYAAGYGIGASLGGFGAAQLIPTFGWRSVFAAGAIATGIATIATFFFLPESVDWLSTRRPAGARDKINYIARRLGKVGTFELPGEQSLSTKKAGLQSYAVLVNKENRGTSIKLWVAFGIVMFGFYFANTWTPKLLVETGMSEQQGIIGGLMLSMGGAFGSLLYGFLTTKFSSRNTLMTFMVLSGLTLILFISSTSVPSIAFASGVVVGMLINGCVAGLYTLSPQLYSAEVRTTGVGAAIGMGRVGAISAPLLVGSLLDSGWSPTQLYVGVAVIVIAGATALIGMRTQAVAVEKQPEALATK

SEQ ID NO: 55 - DNA, 1296 bp, Corynebacterium glutamicum
gtgtcaacgaccaccccaacccgcgcaaccaaaagtgtcggaacagttctcgcactcctgtggttcgcaattgtcctcgacggctttgacctagtcgtcctgggcgcaacaatcccgtccatgctggaggatcccgcgtgggatctcactgctggacaggccacacagatttccaccatcggcctcgtcggcatgaccatcggcgcactgaccattggtttcttaactgaccgtctgggtcgacgccgcgtcatgctgttctctgtggcagtgttttctgtattcaccctcctgctggcattcaccaccaacgtccagctcttcagcctgtggcgtttcctcgcaggtgttggccttggtggagcactccccaccgcaattgccatggtgaccgagtttcgccccggcaccaaagcgggctctgcatcaactaccttgatgaccggataccacgtcggggcagtagcaaccgctttccttggtctcttccttatcgacggctttggttggcactccatgttcatcgcaggcgctgtgccaggactactcctgctgccactgctgtatttcttccttccagaatccccgcagtacctcaaaatctccggcaagttggatgaggcgcaggcagttgcagcatcttatggactttccctggatgatgatcttgatcgcgaacacgaagaagaacttggcgagtcctcctcactttcctccctgttcaagccctcgttccgccgcaacaccctggcgatttggggcacctcattcatgggactcctcctggtctacggcctgaacacatggctgccacaaatcatgcgccaagcagactacgacatgggtaactccctgggcttcctcatggttcttaacatcggcgcagtgatcggcctttatattgcagggcgaattgccgataagaactcccctcgcaaaacagcactcgtatggttcgtgttctctgcatttttcctcgcactacttgctgtccggatgccactgatcggtctgtatggcatcgtgctgctcaccggcatctttgtgttcagctcccaggtactcatctacgccttcgttggtgagaatcaccctgccaagatgcgtgcaactgccatgggattctccgcaggaattggtcgcctcggcgcgatctcgggtccgttgctgggcggcctgcttgtcagtgccaaccttgcttacccatggggcttcttcgccttcgctggcgttggactgctgggcgcgctgattttctccgcatcgaagactctgaggcatcgcgagaacgcttag

SEQ ID NO: 56 - protein, 431 aa, Corynebacterium glutamicum
MSTTTPTRATKSVGTVLALLWFAIVLDGFDLVVLGATIPSMLEDPAWDLTAGQATQISTIGLVGMTIGALTIGFLTDRLGRRRVMLFSVAVFSVFTLLLAFTTNVQLFSLWRFLAGVGLGGALPTAIAMVTEFRPGTKAGSASTTLMTGYHVGAVATAFLGLFLIDGFGWHSMFIAGAVPGLLLLPLLYFFLPESPQYLKISGKLDEAQAVAASYGLSLDDDLDREHEEELGESSSLSSLFKPSFRRNTLAIWGTSFMGLLLVYGLNTWLPQIMRQADYDMGNSLGFLMVLNIGAVIGLYIAGRIADKNSPRKTALVWFVFSAFFLALLAVRMPLIGLYGIVLLTGIFVFSSQVLIYAFVGENHPAKMRATAMGFSAGIGRLGAISGPLLGGLLVSANLAYPWGFFAFAGVGLLGALIFSASKTLRHRENA

SEQ ID NO: 57 - DNA, 1131 bp, Corynebacterium glutamicum
atgacactgtccgaacgcaagctcaccaccaccgccaagattcttccccacccactcaacgcctggtacgtcgccgcttgggattatgaagtcacatctaaaaagcccatggccaggacaatcgccaacaaaccactcgctttgtaccgcaccaaagatggccgagccgttgcccttgcagacgcctgctggcaccgcctcgcaccgctatccaagggaaaactcgtgggcacagacggaatccaatgcccttatcacggcttggagtacaactccgcgggccgctgcatgaaaatgcccgcgcaggaaaccctcaacccgtcagcagccgtcaactcctaccccgtggtggaagcccaccgctttgtgtgggtgtggctgggcgatcccacattggcagatcccacccaagtacccgatatgcaccagatgagccaccccgaatgggcaggcgatggacgcaccatctccgctgactgcaactaccaattagtgctggacaacttgatggacctcacccacgaagaattcgtgcactcctccagcatcggccaagacgaacttagtgaatcagagttcgtggtcacccacactgaagattccgtgacggtcacccgctggatgcatgacatagatgcaccaccgttttggcaaaagaacatgaatgataagttcccaggatttgaaggcaaggtggatcgttggcagatcatccactactactacccttccaccatctgcattgatgttggtgtagcaaaggctggaaccggcgcgcaggaaggcgaccgcagccagggcgttaatgggtatgtaatgaacaccattaccccagattcagatcgttcctctcattacttctgggcattcatgcgcaactaccgcctggaaagccaaaccatcaccacccagctgcgcgacggtgtatccggtgtattcaaagaagacgaagacatgctgaccgctcagcaagatgccatcgacgccaacaccgactatgagttttacagcctcaacattgatgccggtggcatgtgggtgcgccgaatcctcgaggaagcactctccaaggaaggccgactggatatccccaccacattcccccgcgcaacaccgaagccggaggcataa

SEQ ID NO: 58 - protein, 376 aa, Corynebacterium glutamicum
MTLSERKLTTTAKILPHPLNAWYVAAWDYEVTSKKPMARTIANKPLALYRTKDGRAVALADACWHRLAPLSKGKLVGTDGIQCPYHGLEYNSAGRCMKMPAQETLNPSAAVNSYPVVEAHRFVWVWLGDPTLADPTQVPDMHQMSHPEWAGDGRTISADCNYQLVLDNLMDLTHEEFVHSSSIGQDELSESEFVVTHTEDSVTVTRWMHDIDAPPFWQKNMNDKFPGFEGKVDRWQIIHYYYPSTICIDVGVAKAGTGAQEGDRSQGVNGYVMNTITPDSDRSSHYFWAFMRNYRLESQTITTQLRDGVSGVFKEDEDMLTAQQDAIDANTDYEFYSLNIDAGGMWVRRILEEALSKEGRLDIPTTFPRATPKPEA

SEQ ID NO: 59 - DNA, 978 bp, Corynebacterium glutamicum
atgaactcgcaatggcaagatgcacatgttgtttccagcgaaatcatcgctgcagacattcgacgaatagaactatccccgaaatttgcgattccagtaaaacccggcgaacatctcaagatcatggtgcccctaaaaactggacaggaaaagagatcgtactccatcgttgacgctcgtcacgacggttcgactctcgccctgagcgtactcaaaaccagaaactcccgtggaggatctgagttcatgcatacgcttcgagctggagacacagttactgtctccaggccgtctcaggattttcctctccgcgtgggtgcgcctgagtatgtacttgttgccggcggaattggaatcacagcgatccgttcaatggcatctttattaaagaaattgggagcaaactaccgcattcatttcgcagcacgcagccttgatgccatggcttacaaagatgagctcgtggcagaacacggcgacaagctgcacctgcatctagattctgaaggcaccaccatcgatgtcccagcattgatcgaaaccttaaacccccacactgagctttatatgtgcggccccatccgcttgatggatgccatccggcgcgcatggaacacccgcggacttgaccccaccaatctgcgtttcgaaacgtttggaaacagtggatggttctccccagaggttttccacatccaagtaccagagctggggcttcacgccacagtcaacaaggatgaaagcatgctggaggctttgcaaaaggctggggcgaatatgatgtttgattgtcgaaaaggcgaatgtggtttgtgccaggttcgcgttctagaagtcgatggccaggttgatcaccgcgatgtgttcttctctgatcgtcaaaaagaatccgacgcaaaggcatgcgcctgcgtgtctcgagtagtctcctccccttcctcgtccccaacctcgaccattacggtcgccctctcctaa

SEQ ID NO: 60 - protein, 325 aa, Corynebacterium glutamicum
MNSQWQDAHVVSSEIIAADIRRIELSPKFAIPVKPGEHLKIMVPLKTGQEKRSYSIVDARHDGSTLALSVLKTRNSRGGSEFMHTLRAGDTVTVSRPSQDFPLRVGAPEYVLVAGGIGITAIRSMASLLKKLGANYRIHFAARSLDAMAYKDELVAEHGDKLHLHLDSEGTTIDVPALIETLNPHTELYMCGPIRLMDAIRRAWNTRGLDPTNLRFETFGNSGWFSPEVFHIQVPELGLHATVNKDESMLEALQKAGANMMFDCRKGECGLCQVRVLEVDGQVDHRDVFFSDRQKESDAKACACVSRVVSSPSSSPTSTITVALS

SEQ ID NO: 61 - DNA, 615 bp, Corynebacterium glutamicum
atgattgatacagggaagaacggcgagttccgctacgagcagtcgaatatcatcgatcagaacgaagccgagttcggcatcactccttcacagaccgtgggcccttacgtccacatcggtttgacccttgaaggtgcggagcatctcgtggagccaggttcggaaggcgcggtgtcctttactgtttccgcaactgatggcaacggcgaccccatcgcggatgccatgtttgaactgtggcaggccgatccagagggcatccacaactctgatttggatccaaaccgcacagcaccagcaaccgcagatggcttccgcgggcttggtcgcgcgatggcaaacgcgcagggtgaggcaacgttcaccactttggttccgggagcattcgcagatgaggcaccacacttcaaggttggtgtgttcgcccgtggcatgctggagcgtctgtacactcgcgcatacctgccagacgccgatttgagcaccgacccagttttggctgtggtcccagctgatcgacgtgacctcctggtggctcaaaagaccgatgatggattccgcttcgacatcactgtccaggctgaagacaatgaaaccccattttttggactctaa

SEQ ID NO: 62 - protein, 204 aa, Corynebacterium glutamicum
MIDTGKNGEFRYEQSNIIDQNEAEFGITPSQTVGPYVHIGLTLEGAEHLVEPGSEGAVSFTVSATDGNGDPIADAMFELWQADPEGIHNSDLDPNRTAPATADGFRGLGRAMANAQGEATFTTLVPGAFADEAPHFKVGVFARGMLERLYTRAYLPDADLSTDPVLAVVPADRRDLLVAQKTDDGFRFDITVQAEDNETPFFGL

SEQ ID NO: 63 - DNA, 693 bp, Corynebacterium glutamicum
atggacatcccacacttcgccccgacgggaggcgaatactccccactgcacttcccggagtaccggaccaccatcaagcgcaacccaagcaacgatctcatcatggttcctagtcgcctcggcgagtccacgggacctgtcttcggcgaccgcgacttgggagacatcgacaacgacatgaccaaggtgaacggtggcgaggctatcggccagcgcatcttcgttcacggccgtgtcctcggtttcgatggcaagccagttccgcacaccttggtcgaggcgtggcaggcaaacgccgcaggccgttaccgccacaagaatgactcctggccagcgccactggatccacacttcaacggtgttgcacgtactctcaccgacaaggacggccagtaccacttctggaccgttatgccaggtaattacccttggggtaaccaccacaacgcatggcgcccggcgcacattcacttctcgctctatggtcgtcagtttacggagcgtctggtcacccagatgtacttcccgaacgatccattgttcttccaggatccgatctacaacgcggtgccaaagggtgcacgtgagcgcatgatcgcaacgttcgactatgacgagacccgtgaaaacttcgcgcttggttacaagttcgacatcgtccttcgtggccgcaacgccaccccatttgagtaa

SEQ ID NO: 64 - protein, 230 aa, Corynebacterium glutamicum
MDIPHFAPTGGEYSPLHFPEYRTTIKRNPSNDLIMVPSRLGESTGPVFGDRDLGDIDNDMTKVNGGEAIGQRIFVHGRVLGFDGKPVPHTLVEAWQANAAGRYRHKNDSWPAPLDPHFNGVARTLTDKDGQYHFWTVMPGNYPWGNHHNAWRPAHIHFSLYGRQFTERLVTQMYFPNDPLFFQDPIYNAVPKGARERMIATFDYDETRENFALGYKFDIVLRGRNATPFE

SEQ ID NO: 65 - DNA, 1062 bp, Corynebacterium glutamicum
atgagcatccaagtaaaagcactccagaaaaccggccccgaagcacctttcgaggtcaaaatcattgagcgtcgtgagcctcgcgctgacgacgtagttatcgacatcaaagctgccggcatctgccacagcgatatccacaccatccgcaacgaatggggcgaggcacacttcccgctcaccgtcggccacgaaatcgcaggcgttgtctctgcggttggctccgatgtaaccaagtggaaagtcggcgaccgcgttggcgtcggctgcctagttaactcctgcggcgaatgtgaacagtgtgtcgcgggatttgaaaacaactgccttcgcggaaacgtcggaacctacaactccgacgacgtcgacggcaccatcacgcaaggtggctacgccgaaaaggtagtggtcaacgaacgtttcctctgcagcatcccagaggaactcgacttcgatgtcgcagcaccactgctgtgcgcaggcatcaccacctactccccgatcgctcgctggaacgttaaagaaggcgacaaagtagcagtcatgggcctcggcgggctcggccacatgggtgtccaaatcgccgcagccaagggcgctgacgttaccgttctgtcccgttccctgcgcaaggctgaacttgccaaggaactcggcgcagctcgcacgcttgcgacttctgatgaggatttcttcaccgaacacgccggtgaattcgacttcatcctcaacaccattagcgcatccatcccagtcgacaagtacctgagccttctcaagccacacggtgtcatggctgttgtcggtctgccaccagagaagcagccactgagcttcggtgcgctcatcggcggcggaaaagtcctcaccggatccaacattggcggcatccctgaaacccaggaaatgctcgacttctgtgcaaaacacggcctcggcgcgatgatcgaaactgtcggcgtcaacgatgttgatgcagcctacgaccgcgttgttgccggcgacgttcagttccgcgttgtcattgatactgcttcgtttgcagaggtagaggcggtttag

SEQ ID NO: 66 - protein, 353 aa, Corynebacterium glutamicum
MSIQVKALQKTGPEAPFEVKIIERREPRADDVVIDIKAAGICHSDIHTIRNEWGEAHFPLTVGHEIAGVVSAVGSDVTKWKVGDRVGVGCLVNSCGECEQCVAGFENNCLRGNVGTYNSDDVDGTITQGGYAEKVVVNERFLCSIPEELDFDVAAPLLCAGITTYSPIARWNVKEGDKVAVMGLGGLGHMGVQIAAAKGADVTVLSRSLRKAELAKELGAARTLATSDEDFFTEHAGEFDFILNTISASIPVDKYLSLLKPHGVMAVVGLPPEKQPLSFGALIGGGKVLTGSNIGGIPETQEMLDFCAKHGLGAMIETVGVNDVDAAYDRVVAGDVQFRVVIDTASFAEVEAV

SEQ ID NO: 67 - DNA, 1113 bp, Corynebacterium glutamicum
gtgtccatgagcactgtcgtgcctggaattgtcgccctgtccaagggggcaccggtagaaaaagtaaacgttgttgtccctgatccaggtgctaacgatgtcatcgtcaagattcaggcctgcggtgtgtgccacaccgacttggcctaccgcgatggcgatatttcagatgagttcccttacctcctcggccacgaggcagcaggtattgttgaggaggtaggcgagtccgtcacccacgttgaggtcggcgatttcgtcatcttgaactggcgtgcagtgtgcggcgagtgccgtgcatgtaagaagggcgagccaaagtactgctttaacacccacaacgcatctaagaagatgaccctggaagacggcaccgagctgtccccagcactgggtattggcgcgttcttggaaaagaccctggtccacgaaggccagtgcaccaaggttaaccctgaggaagatccagcagcagctggccttctgggttgcggcatcatggcaggtcttggtgctgcggtaaacaccggtgatattaagcgcggcgagtccgtggcagtcttcggccttggtggcgtgggcatggcagctattgctggcgccaagattgctggtgcatcgaagattattgctgttgatatcgatgagaagaagttggagtgggcgaaggaattcggcgcaacccacaccattaattcctctggtcttggtggcgagggtgatgcctctgaggtcgtggcaaaggttcgtgagctcactgatggtttcggtactgacgtctccatcgatgcggtaggcatcatgccgacctggcagcaggcgttttactcccgtgatcatgcaggccgcatggtgatggtgggcgttccaaacctgacgtctcgcgtagatgttcctgcgattgatttttacggtcgcggtggctctgtgcgccctgcatggtacggcgactgcctgcctgagcgtgatttcccaacttatgtggatctgcacctgcagggtcgtttcccgctggataagtttgtttctgagcgtattggtcttgatgatgttgaagaggctttcaacaccatgaaggctggcgacgtgctgcgttctgtggtggagatctaa

SEQ ID NO: 68 - protein, 370 aa, Corynebacterium glutamicum
MSMSTVVPGIVALSKGAPVEKVNVVVPDPGANDVIVKIQACGVCHTDLAYRDGDISDEFPYLLGHEAAGIVEEVGESVTHVEVGDFVILNWRAVCGECRACKKGEPKYCFNTHNASKKMTLEDGTELSPALGIGAFLEKTLVHEGQCTKVNPEEDPAAAGLLGCGIMAGLGAAVNTGDIKRGESVAVFGLGGVGMAAIAGAKIAGASKIIAVDIDEKKLEWAKEFGATHTINSSGLGGEGDASEVVAKVRELTDGFGTDVSIDAVGIMPTWQQAFYSRDHAGRMVMVGVPNLTSRVDVPAIDFYGRGGSVRPAWYGDCLPERDFPTYVDLHLQGRFPLDKFVSERIGLDDVEEAFNTMKAGDVLRSVVEI

SEQ ID NO: 69 - DNA, 1047 bp, Corynebacterium glutamicum
gtgagttttatgaccactgctgcaccccaagaatttaccgctgctgttgttgaaaaattcggtcatgacgtgaccgtgaaggatattgaccttccaaagccagggccacaccaggcattggtgaaggtactcacctccggcatctgccacaccgacctccacgccttggagggcgattggccagtaaagccggaaccaccattcgtaccaggacacgaaggtgtaggtgaagttgttgagctcggaccaggtgaacacgatgtgaaggtcggcgatattgtcggcaatgcgtggctctggtcagcgtgcggcacctgcgaatactgcatcacaggcagggaaactcagtgtaacgaagctgagtacggtggctacacccaaaatggatccttcggccagtacatgctggtggatacccgatacgccgctcgcatcccagacggcgtggactacctcgaagcagcgccaattctgtgtgcaggcgtgactgtctacaaggcactcaaagtctctgaaacccgcccgggccaattcatggtgatctccggtgtcggcggacttggccacatcgcagtccaatacgcagcggcgatgggcatgcgtgtcattgcggtagatattgccgaggacaagctggaacttgcccgtaagcacggtgcggaatttaccgtgaatgcgcgtaatgaagatccaggcgaagctgtacagaagtacaccaacggtggcgcacacggcgtgcttgtgactgcagttcacgaggcagcattcggccaggcactggatatggctcgacgtgcaggaacaattgtgttcaacggtctgccaccgggagagttcccagcatccgtgttcaacatcgtattcaagggcctgaccatccgtggatccctcgtgggaacccgccaagacttggccgaagcgctcgatttctttgcacgcggactaatcaagccaaccgtgagtgagtgctccctcgatgaggtcaatggagttcttgaccgcatgcgaaacggcaagatcgatggtcgtgtggcgattcgtttctaa

SEQ ID NO: 70 - protein, 348 aa, Corynebacterium glutamicum
MSFMTTAAPQEFTAAVVEKFGHDVTVKDIDLPKPGPHQALVKVLTSGICHTDLHALEGDWPVKPEPPFVPGHEGVGEVVELGPGEHDVKVGDIVGNAWLWSACGTCEYCITGRETQCNEAEYGGYTQNGSFGQYMLVDTRYAARIPDGVDYLEAAPILCAGVTVYKALKVSETRPGQFMVISGVGGLGHIAVQYAAAMGMRVIAVDIAEDKLELARKHGAEFTVNARNEDPGEAVQKYTNGGAHGVLVTAVHEAAFGQALDMARRAGTIVFNGLPPGEFPASVFNIVFKGLTIRGSLVGTRQDLAEALDFFARGLIKPTVSECSLDEVNGVLDRMRNGKIDGRVAIRF

SEQ ID NO: 71 - DNA, 1020 bp, Corynebacterium glutamicum
atgcccaaatacattgccatgcaggtatccgaatccggtgcaccgttagccgcgaatctcgtgcaacctgctccgttgaaatcgagggaagtccgcgtggaaatcgctgctagtggtgtgtgccatgcagatattggcacggcagcagcatcggggaagcacactgtttttcctgttacccctggtcatgagattgcaggaaccatcgcggaaattggtgaaaacgtatctcggtggacggttggtgatcgcgttgcaatcggttggtttggtggcaattgcggtgactgcgctttttgtcgtgcaggtgatcctgtgcattgcagagagcggaagattcctggcgtttcttatgcgggtggttgggcacagaatattgttgttccagcggaggctcttgctgcgattccagatggcatggacttttacgaggccgccccgatgggctgcgcaggtgtgacaacattcaatgcgttgcgaaacctgaagctggatcccggtgcggctgtcgcggtctttggaatcggcggtttagtgcgcctagctattcagtttgctgcgaaaatgggttatcgaaccatcaccatcgcccgcggtttagagcgtgaggagctagctaggcaacttggcgccaaccactacatcgatagcaatgatctgcaccctggccaggcgttatttgaacttggcggggctgacttgatcttgtctactgcgtccaccacggagcctctttcggagttgtctaccggtctttctattggcgggcagctaaccattatcggagttgatgggggagatatcaccgtttcggcagcccaattgatgatgaaccgtcagatcatcacaggtcacctcactggaagtgcgaatgacacggaacagactatgaaatttgctcatctccatggcgtgaaaccgcttattgaacggatgcctctcgatcaagccaacgaggctattgcacgtatttcagctggtaaaccacgtttccgtattgtcttggagccgaattcataa

SEQ ID NO: 72 - protein, 339 aa, Corynebacterium glutamicum
MPKYIAMQVSESGAPLAANLVQPAPLKSREVRVEIAASGVCHADIGTAAASGKHTVFPVTPGHEIAGTIAEIGENVSRWTVGDRVAIGWFGGNCGDCAFCRAGDPVHCRERKIPGVSYAGGWAQNIVVPAEALAAIPDGMDFYEAAPMGCAGVTTFNALRNLKLDPGAAVAVFGIGGLVRLAIQFAAKMGYRTITIARGLEREELARQLGANHYIDSNDLHPGQALFELGGADLILSTASTTEPLSELSTGLSIGGQLTIIGVDGGDITVSAAQLMMNRQIITGHLTGSANDTEQTMKFAHLHGVKPLIERMPLDQANEAIARISAGKPRFRIVLEPNS

SEQ ID NO: 73 - DNA, 879 bp, Corynebacterium glutamicum
atgcaaacccttgctgctattgttcgtgccacgaagcaaccttttgagatcaccaccattgatctggatgcaccacgaccagatgaagttcaaatccgtgttattgctgccggagtgcgccacactgacgcaattgttcgtgatcagatttacccaacttttcttcccgcagttttcggccacgaaggcgccggagtagttgtcgccgtgggttctgcagtcacctcggtgaaaccagatgacaaggtagtgctgggattcaactcttgtggccagtgcttgaagtgtttgggcggtaagcctgcgtactgtgagaaattctatgaccgcaacttcgcatgcacccgcgatgccgggcacactactttgtttacccgtgcaacaaaagagcaggcagaggccatcatcgacacccttgatgatgttttctacgatgcggatgcgggtttcctggcatacccagcaactcccccagaggcttcgggagtaagcgtgttggttgtcgcggctggtacctctgatctcccccaagcaaaggaagcactacacactgcctcctacttggggcgctccacctcactgattgttgattttggagtggctggcatccaccgcctgctttcatacgaagaagaactccgcgctgcgggcgtgctcatcgttgccgctggaatggatggtgcgctacccggagttgtcgcaggcttagtgtccgcacctgtcgtcgcactgccaacctccgtgggatacggcgcaggtgctggaggaatcgcaccacttctgaccatgcttaacgcctgcgcgccgggagttggagtggtcaacattgataacggctatggagcaggacacctggctgcgcagattgcggcgaggtaa

SEQ ID NO: 74 - protein, 292 aa, Corynebacterium glutamicum
MQTLAAIVRATKQPFEITTIDLDAPRPDEVQIRVIAAGVRHTDAIVRDQIYPTFLPAVFGHEGAGVVVAVGSAVTSVKPDDKVVLGFNSCGQCLKCLGGKPAYCEKFYDRNFACTRDAGHTTLFTRATKEQAEAIIDTLDDVFYDADAGFLAYPATPPEASGVSVLVVAAGTSDLPQAKEALHTASYLGRSTSLIVDFGVAGIHRLLSYEEELRAAGVLIVAAGMDGALPGVVAGLVSAPVVALPTSVGYGAGAGGIAPLLTMLNACAPGVGVVNIDNGYGAGHLAAQIAAR

SEQ ID NO: 75 - DNA, 3453 bp, Nocardia brasiliensis
ttgttcgccgaggacgagcaggtgaaagccgcggtgccggaccaggaggtggtcgaggcgatccgggcgcccggcctgcgcctggcacagatcatggccaccgtgatggagcgctatgcggaccgccccgcggtgggacagcgggcgagcgagccggtcaccgagagcggtcgcaccaccttccggctgctcccggaattcgagaccctgacctaccgcgagctgtgggcgcgcgtccgcgcggtggccgccgcgtggcacggagatgccgaaaggcctttgcgggccggggatttcgttgctctgctgggtttcgccggcatcgattacggcaccctcgatctcgcgaacatccatctcggcctcgtcacggtgccgctgcaatccggcgccacggccccgcaactcgccgcgatcctggccgagaccacgccccgggtgctggccgcgacacccgaccatctcgatatcgccgtcgaattgctgaccgggggagcctcgccggaacggctggtggtattcgactaccgccccgcggacgacgatcaccgggcggcgctcgagtccgcgcgcagacggttgagcgacgcgggcagtgcggtggtggtcgagacgctcgacgcggtccgcgcccgcggcagcgaattgccggccgcgccgctgttcgttcccgccgcggacgaggacccgctggctctgctcatctacacctccggcagcaccggcacgcctaagggcgccatgtacaccgaaagactgaaccgcacgacgtggctgagcggggcgaaaggcgtcggcctcacgctcggctacatgccgatgagtcatattgccgggcgggcctcgttcgccggtgtgctggcccgcggcggcacggtctacttcaccgcccgcagcgatatgtcgacgctgttcgaagatctggccctggtgcggccgaccgagatgttcttcgtcccgcgcgtgtgcgacatgatcttccagcgctatcaggccgaactgtcgcggcgcgcgcccgccgcggccgcgagcccggaactcgagcaggaactgaagaccgaactgcgcttgtccgcggtcggggaccgcttactcggggcgatcgcgggcagcgcgccgctgtcggccgagatgcgggagttcatggagtcgctgctggatctggaactgcacgacggctacggctcgaccgaggcgggtatcggcgtactgcaagacaatatcgtccagcgtccgccggtcatcgattacaagctcgtcgacgtgccggaattgggctacttccggacggaccagccgcatccccgcggtgagttgctgttgaaaaccgaagggatgattccgggctacttccggcggcccgaggtgaccgcggagatcttcgacgaggacggtttctacaggaccggtgacatcgtcgccgaactcgaaccggatcggctgatctacctggaccgccgcaacaatgtgctgaaactggcccagggcgagttcgtcacggtcgcccatctggaagcggtgttcgcgaccagtccgctgatccggcagatctacatctacggcaacagcgagcgctcgttcctgctggcggtgatcgtgcccaccgcggacgcgctggccgacggtgtcaccgacgcgctgaacacggcgctgaccgaatccttgcgacagctcgcgaaagaagccgggctgcaatcctatgagctgccgcgcgagttcctggtcgaaaccgaaccgttcaccgtcgagaacggtctgctctccggtatcgcgaaactgttgcggcccaagctcaaggagcactacggcgagcgactcgagcagctgtaccgcgatatcgaggcgaaccgcaacgacgagctgatcgagctgcggcgcaccgcggccgagctgccggtgctcgaaaccgtcacgcgggctgcacgttcgatgctcggactggccgcgtcggagttgcggccggacgcgcatttcaccgatctcggcggtgattcactgtccgcgctgtcgttttcgaccctgctgcaggacatgctcgaggtcgaggtcccggtcggtgtcatcgtgagccccgccaactcgctcgccgatctggcgaaatacatcgaggccgaacggcattcgggggtgcggcggccgagcctgatctcggtgcacggtcccggcaccgagatccgtgccgccgatctcaccctggacaagttcatcgacgagcgcaccctcgctgccgcgaaagcggttccggccgcgccggcccaggcgcagaccgtcctgctcaccggggcgaacggctatctcggccgcttcctgtgcctggaatggctgcagcgactggaccagaccggcggcacgctggtctgcatcgtgcgcggtaccgacgcggccgccgcgcggaagcgcctggatgcggtgttcgacagcggtgatccggagctgctcgaccactaccggaagctggccgccgagcacctcgaggtgctcgcgggcgatatcggcgacccgaatctcggcctggacgaagcgacttggcagcggctcgccgcgaccgtcgacctgatcgtgcaccccgccgccctcgtcaaccatgtgctgccgtacagccagctgttcgggccgaatgtggtcggcaccgccgagatcatccggctggccatcaccgagcgccgtaagcccgtgacgtacctgtcgacggtcgcggtggccgcacaggtcgatcccgccggcttcgacgaggagcgcgatatccgggagatgagcgcggtgcgctccatcgacgccgggtacgcgaacggttacggcaacagcaagtgggccggcgaggtgctgctgcgcgaggcccatgatctgtgcgggctgccggtcgccgtgttccgctcggacatgatcctggcgcacagcaaatacgtcggtcagctcaacgtccccgatgtgttcacccggctcatcctgagcctggcgctcaccggcatcgcaccgtattcgttctacgggacggacagcgccgggcagcgcaggcgggcccactacgacggtctgcccgccgatttcgtcgccgaggcgatcaccaccctcggcgcgcgagccgagtcggggttccatacctacgacgtgtggaacccgtacgacgacggcatctcgctggacgaattcgtcgactggctcggcgatttcggcgtgccgatccagcggatcgacgactacgacgaatggttccggcgtttcgagaccgcgatccgcgcgctgcccgaaaagcagcgcgatgcttcgctgctaccgctgctggacgcacaccggcggccactgcgcgcggtgcgcggttcgctgttgcccgccaagaacttccaggcggcggtgcagtccgcgcggatcggccccgatcaggacatcccgcatctttccccgcagttgatcgacaagtacgtcaccgacctgcgccacctcggcctgctctga

SEQ ID NO: 76 - protein, 1150 aa, Nocardia brasiliensis
MFAEDEQVKAAVPDQEVVEAIRAPGLRLAQIMATVMERYADRPAVGQRASEPVTESGRTTFRLLPEFETLTYRELWARVRAVAAAWHGDAERPLRAGDFVALLGFAGIDYGTLDLANIHLGLVTVPLQSGATAPQLAAILAETTPRVLAATPDHLDIAVELLTGGASPERLVVFDYRPADDDHRAALESARRRLSDAGSAVVVETLDAVRARGSELPAAPLFVPAADEDPLALLIYTSGSTGTPKGAMYTERLNRTTWLSGAKGVGLTLGYMPMSHIAGRASFAGVLARGGTVYFTARSDMSTLFEDLALVRPTEMFFVPRVCDMIFQRYQAELSRRAPAAAASPELEQELKTELRLSAVGDRLLGAIAGSAPLSAEMREFMESLLDLELHDGYGSTEAGIGVLQDNIVQRPPVIDYKLVDVPELGYFRTDQPHPRGELLLKTEGMIPGYFRRPEVTAEIFDEDGFYRTGDIVAELEPDRLIYLDRRNNVLKLAQGEFVTVAHLEAVFATSPLIRQIYIYGNSERSFLLAVIVPTADALADGVTDALNTALTESLRQLAKEAGLQSYELPREFLVETEPFTVENGLLSGIAKLLRPKLKEHYGERLEQLYRDIEANRNDELIELRRTAAELPVLETVTRAARSMLGLAASELRPDAHFTDLGGDSLSALSFSTLLQDMLEVEVPVGVIVSPANSLADLAKYIEAERHSGVRRPSLISVHGPGTEIRAADLTLDKFIDERTLAAAKAVPAAPAQAQTVLLTGANGYLGRFLCLEWLQRLDQTGGTLVCIVRGTDAAAARKRLDAVFDSGDPELLDHYRKLAAEHLEVLAGDIGDPNLGLDEATWQRLAATVDLIVHPAALVNHVLPYSQLFGPNVVGTAEIIRLAITERRKPVTYLSTVAVAAQVDPAGFDEERDIREMSAVRSIDAGYANGYGNSKWAGEVLLREAHDLCGLPVAVFRSDMILAHSKYVGQLNVPDVFTRLILSLALTGIAPYSFYGTDSAGQRRRAHYDGLPADFVAEAITTLGARAESGFHTYDVWNPYDDGISLDEFVDWLGDFGVPIQRIDDYDEWFRRFETAIRALPEKQRDASLLPLLDAHRRPLRAVRGSLLPAKNFQAAVQSARIGPDQDIPHLSPQLIDKYVTDLRHLGLL

SEQ ID NO: 77 - DNA, 51 bp, Nocardia brasiliensis
atggcgactgattcgcgaagcgatcggctacggcgtcgaattgcacagttg

SEQ ID NO: 78 - protein, 17 aa, Nocardia brasiliensis
MATDSRSDRLRRRIAQL

SEQ ID NO: 79 - DNA, 3510 bp, Artificial Sequence
  Nucleotide sequence of the DNA-fragment comprising the codon-optimized fadD9 gene and restriction sites
catatggcaactgacagcaggagcgaccgtctacgtaggcggatagctcagctatttgcagaagatgaacaggttaaggcagcagttccggatcaggaagttgttgaagcaattcgtgcacctggtctgcgtctggctcagattatggcaaccgtgatggaacgttacgcagatcgtcctgcagttgggcagcgtgcaagcgaaccggttaccgaaagcgggcgtaccacctttcgtctgttaccggagtttgaaaccctgacctatcgtgaactgtgggcacgtgtgcgtgcagttgcagcagcatggcatggggacgcagagaggcccttacgtgcaggagactttgtcgctctgctggggtttgcaggtattgactatggtaccttagacttagcaaatattcacctgggtttagttaccgttccgctgcaaagcggtgcaactgcaccgcaactggcagcaattctggcagaaaccacccctcgtgttctggcagcaactcctgatcacctggacattgcagtagagctactgaccggaggggcaagcccggagcgtctggttgtctttgactatcgtcctgcagatgatgaccatcgtgcagcattagaaagcgcacgtaggcgtctaagcgatgcaggttcggcagttgttgttgaaaccttagatgcagtccgtgcacgcggtagcgagctaccggcagcaccgctgtttgtccctgcagcagatgaagatccgctggctctgttaatttacaccagcggtagcaccgggacccccaaaggtgcaatgtataccgagaggctgaatcgtactacgtggctgagcggtgcaaagggtgttggtttaaccttaggttatatgccgatgtcgcacatagcaggacgtgcatcatttgcaggggttctggcacgcggtggtaccgtttattttaccgcacgcagcgacatgagcaccctgtttgaggacctggcactggttcgtccgaccgaaatgttttttgttccgcgtgtttgtgacatgatttttcaacgttaccaggcagagctgagccggcgtgcacctgcagcagcagcaagcccggagttagaacaggagctgaaaaccgagctgcgtctaagcgcagtcggagatcgtctattaggggcaattgcaggtagcgcaccgctgagcgcagaaatgcgtgaatttatggaaagcctgctggacctggagctgcatgacggttatggtagcaccgaagcagggattggtgtcctgcaagataacattgttcagaggccgccggttattgactataaattagttgatgttccggagctaggttattttcgtacggatcagccgcaccctcgtggggaactactgctaaagaccgagggaatgataccgggttattttcgtcgtcctgaagttaccgcagaaatttttgacgaagatgggttttacaggaccggggatattgttgcagagttagagccggaccgtctgatttaccttgatcgtcgtaataacgttctgaagctggcacagggtgaatttgttaccgttgcacacctggaggcagtttttgcaacctcgccgctgattcgtcagatttacatttacggtaatagcgaacgtagctttctgctggcagttattgttcctaccgcagatgcactggcagatggggttaccgatgcactgaataccgcactgaccgagagcctaaggcagttagcaaaggaggcaggactgcaaagctacgaactgccgcgtgaatttctggttgagaccgagccgtttaccgtagaaaatgggctgttaagcgggattgcaaagctgctacgtcctaaattaaaagaacattacggtgaaaggttagaacagctgtatcgtgacattgaggcaaatcgtaatgatgaactgattgagctgcgtcgtaccgcagcagaactgccggttttagagaccgtaacccgtgctgctaggagcatgttagggctggcagcaagcgaactacgtccggatgcacactttaccgacttaggtggggactcgctgagcgcactgagcttcagcaccctgctgcaggatatgttagaagttgaagttccggttggggttattgttagccctgcaaatagcttagcagacctggcaaagtatattgaggcagagcgtcacagcggagttcgtcgtccgagcctgattagcgttcatgggcctggtaccgaaattagggcagcagacttaaccctggataaatttattgacgaacgtaccttagctgcagcaaaggcagtcccggcagcaccggcacaggcacagaccgtactgttaaccggagcaaatggttacctgggtcgttttctgtgtctggagtggctgcagaggctggatcagaccggggggaccctggtttgtattgttcgtgggaccgatgcagcagcagcacgcaaacgtctggacgcagtttttgacagcggggacccggagctgttagatcattaccgtaaactggcagcagaacatttagaagttttagcaggtgacattggtgatccgaacttaggtctggatgaggcaacttggcagcgtttagcagcaaccgtcgatctgattgttcatcctgcagcattagttaatcacgttctgccgtatagccagctgtttggaccgaacgttgttggtaccgcagaaattattcgtctggcaattaccgaacgtaggaaacctgttacctatctgagcaccgttgcagttgcagctcaggttgacccggcaggttttgacgaagaacgtgacattcgtgaaatgagcgcagttcgtagcattgacgcaggatatgcaaatgggtatggtaatagcaaatgggcaggtgaagttctgctgcgtgaagcacacgatctgtgtggactgccggttgcagtttttcgtagcgatatgattctggcacatagcaagtatgttgggcagttaaatgttcctgacgtttttacccgtttaattctgagcctggcattaaccgggattgctccgtacagcttttacggaaccgatagcgcaggacagcgtaggcgtgcacattacgacgggctgcctgcagactttgttgcagaagcaattaccaccttaggtgcaagggcagaaagcggatttcacacctatgatgtttggaatccgtatgatgatggtattagcctggatgagtttgttgattggttaggtgactttggtgttccgattcagcgtattgacgactatgatgagtggtttcgtaggtttgaaaccgcaattcgtgcactgcctgagaaacagcgtgacgctagcctgctaccgctgctggatgctcatcgtcgtcccctgcgtgcagttcgtgggagcctgctacctgcaaaaaattttcaagcagcagttcagagcgcacgcattggtcctgaccaggatattccgcacctaagcccgcagctaattgacaaatatgttaccgatctgcgtcatttaggtctgttataagagctc

SEQ ID NO: 80 - DNA, 6557 bp, Artificial Sequence
  Nucleotide sequence of the pELAC vector
tggcgaatgggacgcgccctgtagcggcgcattaagcgcggcgggtgtggtggttacgcgcagcgtgaccgctacacttgccagcgccctagcgcccgctcctttcgctttcttcccttcctttctcgccacgttcgccggctttccccgtcaagctctaaatcgggggctccctttagggttccgatttagtgctttacggcacctcgaccccaaaaaacttgattagggtgatggttcacgtagtgggccatcgccctgatagacggtttttcgccctttgacgttggagtccacgttctttaatagtggactcttgttccaaactggaacaacactcaaccctatctcggtctattcttttgatttataagggattttgccgatttcggcctattggttaaaaaatgagctgatttaacaaaaatttaacgcgaattttaacaaaatattaacgtttacaatttcaggtggcacttttcggggaaatgtgcgcggaacccctatttgtttatttttctaaatacattcaaatatgtatccgctcatgagacaataaccctgataaatgcttcaataatattgaaaaaggaagagtatgagtattcaacatttccgtgtcgcccttattcccttttttgcggcattttgccttcctgtttttgctcacccagaaacgctggtgaaagtaaaagatgctgaagatcagttgggtgcacgagtgggttacatcgaactggatctcaacagcggtaagatccttgagagttttcgccccgaagaacgttttccaatgatgagcacttttaaagttctgctatgtggcgcggtattatcccgtattgacgccgggcaagagcaactcggtcgccgcatacactattctcagaatgacttggttgagtactcaccagtcacagaaaagcatcttacggatggcatgacagtaagagaattatgcagtgctgccataaccatgagtgataacactgcggccaacttacttctgacaacgatcggaggaccgaaggagctaaccgcttttttgcacaacatgggggatcatgtaactcgccttgatcgttgggaaccggagctgaatgaagccataccaaacgacgagcgtgacaccacgatgcctgcagcaatggcaacaacgttgcgcaaactattaactggcgaactacttactctagcttcccggcaacaattaatagactggatggaggcggataaagttgcaggaccacttctgcgctcggcccttccggctggctggtttattgctgataaatctggagccggtgagcgtgggtctcgcggtatcattgcagcactggggccagatggtaagccctcccgtatcgtagttatctacacgacggggagtcaggcaactatggatgaacgaaatagacagatcgctgagataggtgcctcactgattaagcattggtaactgtcagaccaagtttactcatatatactttagattgatttaaaacttcatttttaatttaaaaggatctaggtgaagatcctttttgataatctcatgaccaaaatcccttaacgtgagttttcgttccactgagcgtcagaccccgtagaaaagatcaaaggatcttcttgagatcctttttttctgcgcgtaatctgctgcttgcaaacaaaaaaaccaccgctaccagcggtggtttgtttgccggatcaagagctaccaactctttttccgaaggtaactggcttcagcagagcgcagataccaaatactgtccttctagtgtagccgtagttaggccaccacttcaagaactctgtagcaccgcctacatacctcgctctgctaatcctgttaccagtggctgctgccagtggcgataagtcgtgtcttaccgggttggactcaagacgatagttaccggataaggcgcagcggtcgggctgaacggggggttcgtgcacacagcccagcttggagcgaacgacctacaccgaactgagatacctacagcgtgagctatgagaaagcgccacgcttcccgaagggagaaaggcggacaggtatccggtaagcggcagggtcggaacaggagagcgcacgagggagcttccagggggaaacgcctggtatctttatagtcctgtcgggtttcgccacctctgacttgagcgtcgatttttgtgatgctcgtcaggggggcggagcctatggaaaaacgccagcaacgcggcctttttacggttcctggccttttgctggccttttgctcacatgttctttcctgcgttatcccctgattctgtggataaccgtattaccgcctttgagtgagctgataccgctcgccgcagccgaacgaccgagcgcagcgagtcagtgagcgaggaagcggaagagcgcctgatgcggtattttctccttacgcatctgtgcggtatttcacaccgcatatatggtgcactctcagtacaatctgctctgatgccgcatagttaagccagtatacactccgctatcgctacgtgactgggtcatggctgcgccccgacacccgccaacacccgctgacgcgccctgacgggcttgtctgctcccggcatccgcttacagacaagctgtgaccgtctccgggagctgcatgtgtcagaggttttcaccgtcatcaccgaaacgcgcgaggcagctgcggtaaagctcatcagcgtggtcgtgaagcgattcacagatgtctgcctgttcatccgcgtccagctcgttgagtttctccagaagcgttaatgtctggcttctgataaagcgggccatgttaagggcggttttttcctgtttggtcactgatgcctccgtgtaagggggatttctgttcatgggggtaatgataccgatgaaacgagagaggatgctcacgatacgggttactgatgatgaacatgcccggttactggaacgttgtgagggtaaacaactggcggtatggatgcggcgggaccagagaaaaatcactcagggtcaatgccagcgcttcgttaatacagatgtaggtgttccacagggtagccagcagcatcctgcgatgcagatccggaacataatggtgcagggcgctgacttccgcgtttccagactttacgaaacacggaaaccgaagaccattcatgttgttgctcaggtcgcagacgttttgcagcagcagtcgcttcacgttcgctcgcgtatcggtgattcattctgctaaccagtaaggcaaccccgccagcctagccgggtcctcaacgacaggagcacgatcatgcgcacccgtggggccgccatgccggcgataatggcctgcttctcgccgaaacgtttggtggcgggaccagtgacgaaggcttgagcgagggcgtgcaagattccgaataccgcaagcgacaggccgatcatcgtcgcgctccagcgaaagcggtcctcgccgaaaatgacccagagcgctgccggcacctgtcctacgagttgcatgataaagaagacagtcataagtgcggcgacgatagtcatgccccgcgcccaccggaaggagctgactgggttgaaggctctcaagggcatcggtcgagatcccggtgcctaatgagtgagctaacttacattaattgcgttgcgctcactgcccgctttccagtcgggaaacctgtcgtgccagctgcattaatgaatcggccaacgcgcggggagaggcggtttgcgtattgggcgccagggtggtttttcttttcaccagtgagacgggcaacagctgattgcccttcaccgcctggccctgagagagttgcagcaagcggtccacgctggtttgccccagcaggcgaaaatcctgtttgatggtggttaacggcgggatataacatgagctgtcttcggtatcgtcgtatcccactaccgagatatccgcaccaacgcgcagcccggactcggtaatggcgcgcattgcgcccagcgccatctgatcgttggcaaccagcatcgcagtgggaacgatgccctcattcagcatttgcatggtttgttgaaaaccggacatggcactccagtcgccttcccgttccgctatcggctgaatttgattgcgagtgagatatttatgccagccagccagacgcagacgcgccgagacagaacttaatgggcccgctaacagcgcgatttgctggtgacccaatgcgaccagatgctccacgcccagtcgcgtaccgtcttcatgggagaaaataatactgttgatgggtgtctggtcagagacatcaagaaataacgccggaacattagtgcaggcagcttccacagcaatggcatcctggtcatccagcggatagttaatgatcagcccactgacgcgttgcgcgagaagattgtgcaccgccgctttacaggcttcgacgccgcttcgttctaccatcgacaccaccacgctggcacccagttgatcggcgcgagatttaatcgccgcgacaatttgcgacggcgcgtgcagggccagactggaggtggcaacgccaatcagcaacgactgtttgcccgccagttgttgtgccacgcggttgggaatgtaattcagctccgccatcgccgcttccactttttcccgcgttttcgcagaaacgtggctggcctggttcaccacgcgggaaacggtctgataagagacaccggcatactctgcgacatcgtataacgttactggtttcacattcaccaccctgaattgactctcttccgggcgctatcatgccataccgcgaaaggttttgcgccattcgatggtgtccgggatctcgacgctctcccttatgcgactcctgcattaggaagcagcccagtagtaggttgaggccgttgagcaccgccgccgcaaggaatggtgcatgcaaggagatggcgcccaacagtcccccggccacggggcctgccaccatacccacgccgaaacaagcgctcatgagcccgaagtggcgagcccgatcttccccatcggtgatgtcggcgatataggcgccagcaaccgcacctgtggcgccggtgatgccggccacgatgcgtccggcgtagaggatcgagatctgcgggcagtgagcgcaacgcaattaatgtgagttagctcactcattaggcaccccaggctttacactttatgcttccggctcgtataatgtgtggaattgtgagcggataacaatttcacacaggatctagatttaagaaggagatatacatatggccgaagaaggtaaactggtaatctggattaacggcgataaaggctataacggtctcgctgaagtcggtaagaaattcgagaaagataccggaattaaagtcaccgttgagcatccggataaactggaagagaaattcccacaggttgcggcaacaggcgatggccctgacattatcttctgggcacacgaccgctttggtggctacgctcaatctggcctgttggctgaaatcaccccggacaaagcgttccaggacaagctgtatccgtttacctgggatgccgtacgttacaacggcaagctgattgcttacccgatcgctgttgaagcgttatcgctgatttataacaaagatctgctgccgaacccgccaaaaacctgggaagagatcccggcgctggataaagaactgaaagcgaaaggtaagagcgcgctgatgttcaacctgcaagaaccgtacttcacctggccgctgattgctgctgacgggggttatgcgttcaagtatgaaaacggcaagtacgacattaaagacgtgggcgtggataacgctggcgcgaaagcgggtctgaccttcctggttgacctgattaaaaacaaacacatgaatgcagacaccgattactccatcgcagaagctgcctttaataaaggcgaaacagcgatgaccatcaacggcccgtgggcatggtccaacatcgacaccagcaaagtgaattatggtgtaacggtactgccgaccttcaagggtcaaccatccaaaccgttcgttggcgtgctgagcgcaggtattaacgccgccagtccgaacaaagagctggcaaaagagttcctcgaaaactatctgctgactgatgaaggtctggaagcggttaataaagacaaaccgctgggtgccgtagcgctgaagtcttacgaggaagagttggcgaaagatccacgtattgccgccactatggaaaacgcccagaaaggtgaaatcatgccgaacatcccgcagatgtccgctttctggtatgccgtgcgtactgcggtgatcaacgccgccagcggtcgtcagactgtcgatgaagccctgaaagacgcgcagactaaggatccgaattcgagctccgtcgacaagcttgcggccgcactcgagcaccaccaccaccaccactgagatccggctgctaacaaagcccgaaaggaagctgagttggctgctgccaccgctgagcaataactagcataaccccttggggcctctaaacgggtcttgaggggttttttgctgaaaggaggaactatatccggat

SEQ ID NO: 81 - DNA, 17 bp, Artificial Sequence
  Primer P1
cgtggctggcctggttc

SEQ ID NO: 82 - DNA, 19 bp, Artificial Sequence
  Primer P5
cgtccccatgccatgctgc

SEQ ID NO: 83 - DNA, 20 bp, Artificial Sequence
  Primer P4
cgctgttgagatccagttcg

SEQ ID NO: 84 - DNA, 19 bp, Artificial Sequence
  Primer P6
gcacattacgacgggctgc

SEQ ID NO: 85 - DNA, 1053 bp, Escherichia coli
atgaattatcagaacgacgatttacgcatcaaagaaatcaaagagttacttcctcctgtcgcattgctggaaaaattccccgctactgaaaatgccgcgaatacggttgcccatgcccgaaaagcgatccataagatcctgaaaggtaatgatgatcgcctgttggttgtgattggcccatgctcaattcatgatcctgtcgcggcaaaagagtatgccactcgcttgctggcgctgcgtgaagagctgaaagatgagctggaaatcgtaatgcgcgtctattttgaaaagccgcgtaccacggtgggctggaaagggctgattaacgatccgcatatggataatagcttccagatcaacgacggtctgcgtatagcccgtaaattgctgcttgatattaacgacagcggtctgccagcggcaggtgagtttctcgatatgatcaccccacaatatctcgctgacctgatgagctggggcgcaattggcgcacgtaccaccgaatcgcaggtgcaccgcgaactggcatcagggctttcttgtccggtcggcttcaaaaatggcaccgacggtacgattaaagtggctatcgatgccattaatgccgccggtgcgccgcactgcttcctgtccgtaacgaaatgggggcattcggcgattgtgaataccagcggtaacggcgattgccatatcattctgcgcggcggtaaagagcctaactacagcgcgaagcacgttgctgaagtgaaagaagggctgaacaaagcaggcctgccagcacaggtgatgatcgatttcagccatgctaactcgtccaaacaattcaaaaagcagatggatgtttgtgctgacgtttgccagcagattgccggtggcgaaaaggccattattggcgtgatggtggaaagccatctggtggaaggcaatcagagcctcgagagcggggagccgctggcctacggtaagagcatcaccgatgcctgcatcggctgggaagataccgatgctctgttacgtcaactggcgaatgcagtaaaagcgcgtcgcgggtaa

SEQ ID NO: 86 - protein, 350 aa, Escherichia coli
MNYQNDDLRIKEIKELLPPVALLEKFPATENAANTVAHARKAIHKILKGNDDRLLVVIGPCSIHDPVAAKEYATRLLALREELKDELEIVMRVYFEKPRTTVGWKGLINDPHMDNSFQINDGLRIARKLLLDINDSGLPAAGEFLDMITPQYLADLMSWGAIGARTTESQVHRELASGLSCPVGFKNGTDGTIKVAIDAINAAGAPHCFLSVTKWGHSAIVNTSGNGDCHIILRGGKEPNYSAKHVAEVKEGLNKAGLPAQVMIDFSHANSSKQFKKQMDVCADVCQQIAGGEKAIIGVMVESHLVEGNQSLESGEPLAYGKSITDACIGWEDTDALLRQLANAVKARRG

SEQ ID NO: 87 - DNA, 1089 bp, Escherichia coli
atggagaggattgtcgttactctcggggaacgtagttacccaattaccatcgcatctggtttgtttaatgaaccagcttcattcttaccgctgaaatcgggcgagcaggtcatgttggtcaccaacgaaaccctggctcctctgtatctcgataaggtccgcggcgtacttgaacaggcgggtgttaacgtcgatagcgttatcctccctgacggcgagcagtataaaagcctggctgtactcgataccgtctttacggcgttgttacaaaaaccgcatggtcgcgatactacgctggtggcgcttggcggcggcgtagtgggcgatctgaccggcttcgcggcggcgagttatcagcgcggtgtccgtttcattcaagtcccgacgacgttactgtcgcaggtcgattcctccgttggcggcaaaactgcggtcaaccatcccctcggtaaaaacatgattggcgcgttctaccaacctgcttcagtggtggtggatctcgactgtctgaaaacgcttcccccgcgtgagttagcgtcggggctggcagaagtcatcaaatacggcattattcttgacggtgcgttttttaactggctggaagagaatctggatgcgttgttgcgtctggacggtccggcaatggcgtactgtattcgccgttgttgtgaactgaaggcagaagttgtcgccgccgacgagcgcgaaaccgggttacgtgctttactgaatctgggacacacctttggtcatgccattgaagctgaaatggggtatggcaattggttacatggtgaagcggtcgctgcgggtatggtgatggcggcgcggacgtcggaacgtctcgggcagtttagttctgccgaaacgcagcgtattataaccctgctcaagcgggctgggttaccggtcaatgggccgcgcgaaatgtccgcgcaggcgtatttaccgcatatgctgcgtgacaagaaagtccttgcgggagagatgcgcttaattcttccgttggcaattggtaagagtgaagttcgcagcggcgtttcgcacgagcttgttcttaacgccattgccgattgtcaatcagcgtaa

SEQ ID NO: 88 - protein, 362 aa, Escherichia coli
MERIVVTLGERSYPITIASGLFNEPASFLPLKSGEQVMLVTNETLAPLYLDKVRGVLEQAGVNVDSVILPDGEQYKSLAVLDTVFTALLQKPHGRDTTLVALGGGVVGDLTGFAAASYQRGVRFIQVPTTLLSQVDSSVGGKTAVNHPLGKNMIGAFYQPASVVVDLDCLKTLPPRELASGLAEVIKYGIILDGAFFNWLEENLDALLRLDGPAMAYCIRRCCELKAEVVAADERETGLRALLNLGHTFGHAIEAEMGYGNWLHGEAVAAGMVMAARTSERLGQFSSAETQRIITLLKRAGLPVNGPREMSAQAYLPHMLRDKKVLAGEMRLILPLAIGKSEVRSGVSHELVLNAIADCQSA

SEQ ID NO: 89 - DNA, 759 bp, Escherichia coli
atgaaaaccgtaactgtaaaagatctcgtcattggtacgggcgcacctaaaatcatcgtctcgctgatggcgaaagatatcgccagcgtgaaatccgaagctctcgcctatcgtgaagcggactttgatattctggaatggcgtgtggaccactatgccgacctctccaatgtggagtctgtcatggcggcagcaaaaattctccgtgagaccatgccagaaaaaccgctgctgtttaccttccgcagtgccaaagaaggcggcgagcaggcgatttccaccgaggcttatattgcactcaatcgtgcagccatcgacagcggcctggttgatatgatcgatctggagttatttaccggtgatgatcaggttaaagaaaccgtcgcctacgcccacgcgcatgatgtgaaagtagtcatgtccaaccatgacttccataaaacgccggaagccgaagaaatcattgcccgtctgcgcaaaatgcaatccttcgacgccgatattcctaagattgcgctgatgccgcaaagtaccagcgatgtgctgacgttgcttgccgcgaccctggagatgcaggagcagtatgccgatcgtccaattatcacgatgtcgatggcaaaaactggcgtaatttctcgtctggctggtgaagtatttggctcggcggcaacttttggtgcggtaaaaaaagcgtctgcgccagggcaaatctcggtaaatgatttgcgcacggtattaactattttacaccaggcataa

SEQ ID NO: 90 - protein, 252 aa, Escherichia coli
MKTVTVKDLVIGTGAPKIIVSLMAKDIASVKSEALAYREADFDILEWRVDHYADLSNVESVMAAAKILRETMPEKPLLFTFRSAKEGGEQAISTEAYIALNRAAIDSGLVDMIDLELFTGDDQVKETVAYAHAHDVKVVMSNHDFHKTPEAEEIIARLRKMQSFDADIPKIALMPQSTSDVLTLLAATLEMQEQYADRPIITMSMAKTGVISRLAGEVFGSAATFGAVKKASAPGQISVNDLRTVLTILHQA

SEQ ID NO: 91 - DNA, 843 bp, Bacillus thuringiensis
atgaaatattcgctatgtaccatttcatttcgtcatcaattaatttcatttactgatattgttcaatttgcatatgaaaacggttttgaaggaattgaattatgggggacgcatgcacaaaatttgtacatgcaagaacgtgaaacgacagaacgagaattgaattttctaaaggataaaaacttagaaattacgatgataagtgattacttagatatatcattatcagcagattttgaaaaaacgatagagaaaagtgaacaacttgtagtactagctaattggtttaatacgaataaaattcgcacgtttgctgggcaaaaagggagcaaggacttctcggaacaagagagaaaagagtatgtgaagcgaatacgtaagatttgtgatgtgtttgctcagaacaatatgtatgtgctgttagaaacacatcccaatacactaacggacacattgccttctactatagagttattagaagaagtaaaccatccgaatttaaaaataaatcttgattttcttcatatatgggagtctggcgcagatccaatagacagtttccatcgattaaagccgtggacactacattaccattttaagaatatatcttcagcggattatttgcatgtgtttgaacctaataatgtatatgctgcagcaggaagtcgtataggtatggttccgttatttgaaggtattgtaaattatgatgagattattcaggaagtgagaaatacggatctttttgcttccttagaatggtttggacataattcaaaagagatattaaaagaagaaatgaaagtattaataaatagaaaattagaagtagtaacttcgtaa

SEQ ID NO: 92 - protein, 280 aa, Bacillus thuringiensis
MKYSLCTISFRHQLISFTDIVQFAYENGFEGIELWGTHAQNLYMQERETTERELNFLKDKNLEITMISDYLDISLSADFEKTIEKSEQLVVLANWFNTNKIRTFAGQKGSKDFSEQERKEYVKRIRKICDVFAQNNMYVLLETHPNTLTDTLPSTIELLEEVNHPNLKINLDFLHIWESGADPIDSFHRLKPWTLHYHFKNISSADYLHVFEPNNVYAAAGSRIGMVPLFEGIVNYDEIIQEVRNTDLFASLEWFGHNSKEILKEEMKVLINRKLEVVTS

SEQ ID NO: 93 - DNA, 1542 bp, Escherichia coli
atgcgtctggaagtcttttgtgaagaccgactcggtctgacccgcgaattactcgatctactcgtgctaagaggcattgatttacgcggtattgagattgatcccattgggcgaatctacctcaattttgctgaactggagtttgagagtttcagcagtctgatggccgaaatacgccgtattgcgggtgttaccgatgtgcgtactgtcccgtggatgccttccgaacgtgagcatctggcgttgagcgcgttactggaggcgttgcctgaacctgtgctctctgtcgatatgaaaagcaaagtggatatggcgaacccggcgagctgtcagctttttgggcaaaaattggatcgcctgcgcaaccataccgccgcacaattgattaacggctttaattttttacgttggctggaaagcgaaccgcaagattcgcataacgagcatgtcgttattaatgggcagaatttcctgatggagattacgcctgtttatcttcaggatgaaaatgatcaacacgtcctgaccggtgcggtggtgatgttgcgatcaacgattcgtatgggccgccagttgcaaaatgtcgccgcccaggacgtcagcgccttcagtcaaattgtcgccgtcagcccgaaaatgaagcatgttgtcgaacaggcgcagaaactggcgatgctaagcgcgccgctgctgattacgggtgacacaggtacaggtaaagatctctttgcctacgcctgccatcaggcaagccccagagcgggcaaaccttacctggcgctgaactgtgcgtctataccggaagatgcggtcgagagtgaactgtttggtcatgctccggaagggaagaaaggattctttgagcaggcgaacggtggttcggtgctgttggatgaaataggggaaatgtcaccacggatgcaggcgaaattactgcgtttccttaatgatggcactttccgtcgggttggcgaagaccatgaggtgcatgtcgatgtgcgggtgatttgcgctacgcagaagaatctggtcgaactggtgcaaaaaggcatgttccgtgaagatctctattatcgtctgaacgtgttgacgctcaatctgccgccgctacgtgactgtccgcaggacatcatgccgttaactgagctgttcgtcgcccgctttgccgacgagcagggcgtgccgcgtccgaaactggccgctgacctgaatactgtacttacgcgttatgcgtggccgggaaatgtgcggcagttaaagaacgctatctatcgcgcactgacacaactggacggttatgagctgcgtccacaggatattttgttgccggattatgacgccgcaacggtagccgtgggcgaagatgcgatggaaggttcgctggacgaaatcaccagccgttttgaacgctcggtattaacccagctttatcgcaattatcccagcacgcgcaaactggcaaaacgtctcggcgtttcacataccgcgattgccaataagttgcgggaatatggtctgagtcagaagaagaacgaagagtaa

SEQ ID NO: 94 - protein, 513 aa, Escherichia coli
MRLEVFCEDRLGLTRELLDLLVLRGIDLRGIEIDPIGRIYLNFAELEFESFSSLMAEIRRIAGVTDVRTVPWMPSEREHLALSALLEALPEPVLSVDMKSKVDMANPASCQLFGQKLDRLRNHTAAQLINGFNFLRWLESEPQDSHNEHVVINGQNFLMEITPVYLQDENDQHVLTGAVVMLRSTIRMGRQLQNVAAQDVSAFSQIVAVSPKMKHVVEQAQKLAMLSAPLLITGDTGTGKDLFAYACHQASPRAGKPYLALNCASIPEDAVESELFGHAPEGKKGFFEQANGGSVLLDEIGEMSPRMQAKLLRFLNDGTFRRVGEDHEVHVDVRVICATQKNLVELVQKGMFREDLYYRLNVLTLNLPPLRDCPQDIMPLTELFVARFADEQGVPRPKLAADLNTVLTRYAWPGNVRQLKNAIYRALTQLDGYELRPQDILLPDYDAATVAVGEDAMEGSLDEITSRFERSVLTQLYRNYPSTRKLAKRLGVSHTAIANKLREYGLSQKKNEE

SEQ ID NO: 95 - DNA, 666 bp, Niastella koreensis
atgaataatcaaatttttgaatccgttgaccattatatcagcgatttactgggttacgaagacgatgcattgcttgccgccaccaattcattagccgaagcaggcatgcctgccatcagcgtatcacccaaccagggcaagtttctgcaattactggcccaattgtgccaggcaaaaaatatcctggagctgggcacactggcaggctacagcaccatttggatggcccgggccttacccaaaaacggccggctcatcacccttgaatatgaccccaaacatgcggccgttgcacaaaaaaatatcgaccgggccggccttacttcacaagtacagatcagaaccggtaaagcaattgacatattaccgcaattagtggaagaaggcgccggaccttttgatatgatctttatcgatgccgataaaccaccttacaccgaatattttcaatgggcgcttcggttatcacgtcccggtacactcatcgtggccgataatgtgatccgtgatggcaaagtgctggatgaaaacagtacggagcctgctgtacagggcgcaagacgtttcaatgccatgctgggcgccaataccgccgttgacgccaccattcttcaaatggtaggtgtaaaagaatacgatggaatggctttggccatagtaaaataa

SEQ ID NO: 96 - protein, 221 aa, Niastella koreensis
MNNQIFESVDHYISDLLGYEDDALLAATNSLAEAGMPAISVSPNQGKFLQLLAQLCQAKNILELGTLAGYSTIWMARALPKNGRLITLEYDPKHAAVAQKNIDRAGLTSQVQIRTGKAIDILPQLVEEGAGPFDMIFIDADKPPYTEYFQWALRLSRPGTLIVADNVIRDGKVLDENSTEPAVQGARRFNAMLGANTAVDATILQMVGVKEYDGMALAIVK

SEQ ID NO: 97 - DNA, 3387 bp, Gordonia effusa
atgtctgaccagcccaacgcgcttccgtctgccatcgagccgctgaaccccgatcctcaagcgacagagcagatctcgcactgtgcgacgattgccgaacttgtccgggttctcgccgagagctacggtgatcgccccgcgctgggttggcgaaacaatagtgatccctcgtcctggcattcgatgacttaccgagatctcgctgagcgggcggattccatggcgcgacttctccattcgacacttggcgtcgccgagaacgaccgggtggcgacggtgggcttcactagcgcggagtacaccatcgcctcgcttgccgtcggcacgctcggcgcgatggaggtaccactgcaaaacgccgggtccgtcgacgtctgggccgcaatcctcaccgaaaccgactgtgtgagcgcggttgtcgcggccgatcaactgccttcgatcgctcggctggccgaatcgggcacctacaccggcctgcgacatgtgctggtcttcgacatcggctcgcgcgacggaaccacgctcgatgacgcggcacgacgactggtcgctgcgggcacccaggtgcatctccgccagcccggcgccgagccgacgacaccgccggctccactgccccagatcacggccaaccccgaccgcgtcgccctcctcatctacacctccggtagcaccggagcccccaaaggcgccatgtacaccgaaaccgcggtgacccggttattccaatcgggactcagcggcttggggcgcgccaccgacggtcacggctggatcaccctgaacttcatgccgatgagccacgtgatgggacgcagcactctgtggcaaaccctgggaaatggtggcaccgcgtacttcaccccgcgcgccgacctcgccgagttgctcaccgacctcgcagcggtccagccgaccgacctgcaattcgtaccgcgcatctgggacatgctgtaccaggagtacgtccgcctcaccgatcaggacgtcagtgaacaagacgccctcacccgtatgcgcgaacactatttcggtacccggactgccaccgccatcaccggttccgcaccgatctccgatgaggttcggcgtttcgtcgaagcgatgctgccggttccactcatcgaaggctatggaagtaccgaggccgccggcgtctccatcgacggccgcatccagcgaccgccggtggtggattacaagcttctcgacgttcctgaactcggctacctgagcaccgatcggccgcacccgcgcggcgaactgctcgtcaagaccgaccatatcttcgcggggtactacaaccgtcccgacctcacctcatcggtcttcgacgaccagggctactaccggacgggcgacatcgtcgccgagaccggcccagaccaaatcgagtatgtcgaccgccggaacaacgtgatgaagctttcgcagggtgagttcgtcgcgatcgcccacatcgaggcggtactgaccaccccgccgatccagcaactgtacgtctacggcaacagcgcgcggccctatctgctcgcggtcgtcgtgcccacccccgagttacgcgaacgacacgccgacgacaacgagctgcgacgagaagtactgacggcactgcgctctcatggcgaacgtaatggccttgcggccgtagagattccgcgcgatgtgattgtcgaacgcacgccgttcagcctggagaacggtcttcttaccggcatccgaaaactcgcgcgcccacaactcaaagagcgctacggcgctcggctggaggccctctacgccgagctggccgatagccgtatcaccaggctgcgcgacgtcaaagccgttgccgcacaacgctcaacggtgacaacggtcatcgacgtggtcacagcgatactcgacctcgccgacggggaggtcacggccgcggcacatttcaccgacctcggcggagattccctcaccgccgtcacggtcgggaacgaactccgcgacatcttcgacgccgaagtaccggtcggcgtcttgaccagcccgtcatcgacgctggccgacatagccgaacatatcgacgggcgacacagcgaggcccggccaaccgcggaatcggtccacggcaccggaaccacccttcgggcagcggacctcactctcgacaaattcctcgacgaggagaccttgcgcgctgcgtccgacgtgacgtcggctgcgaccgacgtacggaccgtattcatcaccggcgcaaccggattcctcggtcgctatctgacactcgactggttgcgtcggatggcaaaagtcggcggcacggtgatctgcctcgttcgaggtgcggacgatgatgccgcccgggcgcgcctagacgcggcattcgactccagcgatctatggtcggagtaccagcgactggccaaagaccaccttcgggttctcgccggcgacaaggactcggatcacctcgcgctcaccccagacgtatgggatgaattggcaaagtccgtcgacctcatcatcgatcccgcggcgctggtcaaccatgtgttgccatatcgagaactattcggacccaacgtatctggcactgctgagctgatcagactcgcggtgacgaccacccgtaagccatacgtgtatatctcaacggtcggtgtaggcgaccaggtcgcgccgggatctttcaccgaggaccccgacatccgcgagatgagctcggtacgcgagattaacgacacttacgccaacggatatggcaacagcaaatgggccggcgaagtattgctcgcgcaggcgcacgaacgatttgagttaccggtcagcgtctttcgctgcgacatgatcgtcgccgatgatcacaccatcgggcagctgaacctacctgacatgttcacgcggctactgatgagcgtgctcgccaccggcttggcacctcgctctttctatcaactcgccaccgacggatcggcacaggaggcccacttcgatgctctgccggtcgatttcctcgccgaagcgatcaacaccctgtgggttaaggacggagcccgcaccttcaacgcgatgaacccgcacgccgacggcatcggattcgatcagtacattcgctggctgatcgacagcggcgagcagatcagccttgtagacaactatgacgattggtatcggcgattcggtgcggccctcgccgatctgccggaaaagcagcgacgcggatcgttgattccgttgctgcacaactatgttcacccgatgacgccgcacaatcgcggtatggcgtcggcggaccgattccacgacgcggtccgaaccgctggcgtcgggcagtcgtccgacatcccgcatatcacgccacagatcatcgagaactacgcccgcagcctccgcggtctcggggtgatctga

SEQ ID NO: 98 - protein, 1128 aa, Gordonia effusa
MSDQPNALPSAIEPLNPDPQATEQISHCATIAELVRVLAESYGDRPALGWRNNSDPSSWHSMTYRDLAERADSMARLLHSTLGVAENDRVATVGFTSAEYTIASLAVGTLGAMEVPLQNAGSVDVWAAILTETDCVSAVVAADQLPSIARLAESGTYTGLRHVLVFDIGSRDGTTLDDAARRLVAAGTQVHLRQPGAEPTTPPAPLPQITANPDRVALLIYTSGSTGAPKGAMYTETAVTRLFQSGLSGLGRATDGHGWITLNFMPMSHVMGRSTLWQTLGNGGTAYFTPRADLAELLTDLAAVQPTDLQFVPRIWDMLYQEYVRLTDQDVSEQDALTRMREHYFGTRTATAITGSAPISDEVRRFVEAMLPVPLIEGYGSTEAAGVSIDGRIQRPPVVDYKLLDVPELGYLSTDRPHPRGELLVKTDHIFAGYYNRPDLTSSVFDDQGYYRTGDIVAETGPDQIEYVDRRNNVMKLSQGEFVAIAHIEAVLTTPPIQQLYVYGNSARPYLLAVVVPTPELRERHADDNELRREVLTALRSHGERNGLAAVEIPRDVIVERTPFSLENGLLTGIRKLARPQLKERYGARLEALYAELADSRITRLRDVKAVAAQRSTVTTVIDVVTAILDLADGEVTAAAHFTDLGGDSLTAVTVGNELRDIFDAEVPVGVLTSPSSTLADIAEHIDGRHSEARPTAESVHGTGTTLRAADLTLDKFLDEETLRAASDVTSAATDVRTVFITGATGFLGRYLTLDWLRRMAKVGGTVICLVRGADDDAARARLDAAFDSSDLWSEYQRLAKDHLRVLAGDKDSDHLALTPDVWDELAKSVDLIIDPAALVNHVLPYRELFGPNVSGTAELIRLAVTTTRKPYVYISTVGVGDQVAPGSFTEDPDIREMSSVREINDTYANGYGNSKWAGEVLLAQAHERFELPVSVFRCDMIVADDHTIGQLNLPDMFTRLLMSVLATGLAPRSFYQLATDGSAQEAHFDALPVDFLAEAINTLWVKDGARTFNAMNPHADGIGFDQYIRWLIDSGEQISLVDNYDDWYRRFGAALADLPEKQRRGSLIPLLHNYVHPMTPHNRGMASADRFHDAVRTAGVGQSSDIPHITPQIIENYARSLRGLGVI

SEQ ID NO: 99 - DNA, 4522 bp, Artificial Sequence
  Nucleotide sequence of DNA fragment containing ACAR gene of Gordonia effusa (codon-optimized) and entD gene of Escherichia coli
ccaagcttgcatgccagatcgtttagatccgaaggaaaacgtcgaaaagcaatttgcttttcgacgccccaccccgcgcgttttagcgtgtcagtagacgcgtagggtaagtggggtagcggcttgttagatatcttgaaatcggctttcaacagcattgatttcgatgtatttagctggccgtttgagacgcgatgtccacagggtagctggtagtttgaaaatcaacgccgttgcccttaggattcagtaactggcacattttgtaatgcgctagatctgtgtgcccagtcttccaggctgcttatcacagtgaaagcaaaaccaattcgtggctgcgaaagtcgtagccaccacgaagtccaggaggacatacaatgagcgatcagccgaatgcactgccgagcgcaattgaaccgctgaatccggatccgcaggcaaccgagcagattagccattgtgcaaccattgcagaactggttcgtgttctggcagaaagctatggtgatcgtccggcactgggttggcgtaataatagcgatccgagcagctggcatagcatgacctatcgtgatctggccgaacgtgcagatagcatggcacgtctgctgcatagcaccctgggtgttgcagaaaatgatcgtgttgcaaccgttggttttaccagcgcagaatataccattgcaagcctggcagttggtacactgggtgcaatggaagttccgctgcagaatgcaggtagcgttgatgtttgggcagcaattctgaccgaaaccgattgtgttagcgcagttgttgcagcagatcagctgccgagcattgcccgtctggcggaaagcggcacctataccggtctgcgtcatgttctggtttttgatattggtagccgtgatggcaccaccctggatgatgcagcacgtcgtctggttgccgcaggcacccaggttcatctgcgtcagcctggtgcagaaccgaccacccctccggcaccgctgccgcagattaccgcaaacccggatcgtgtggcactgctgatttataccagcggtagcacaggtgcaccgaaaggtgcaatgtataccgaaacagcagttacccgtctgtttcagagcggtctgagtggtctgggtcgtgcaaccgatggtcatggttggattaccctgaactttatgccgatgagccatgttatgggtcgtagtaccctgtggcagaccctgggtaatggtggcaccgcatattttacaccgcgtgcagatctggctgaactgctgaccgatctggcagccgttcagccgacggatctgcagtttgttccgcgtatttgggatatgctgtatcaagaatatgttcgtctgacagatcaggatgttagcgaacaggatgcactgacccgtatgcgtgaacattatttcggcacccgtaccgcaaccgcaattaccggtagcgcaccgattagtgatgaagttcgtcgttttgttgaagcaatgctgccggttccgctgattgaaggttatggtagcaccgaagcagccggtgttagcattgatggtcgtattcagcgtccgcctgttgttgattataaactgctggatgtgccggaactgggttatctgagcaccgatcgtccgcatccgcgtggtgagctgctggttaaaaccgatcatatttttgccggttattacaatcgtccggatctgaccagcagcgtttttgatgatcagggttattatcgtaccggtgatattgttgccgaaaccggtccggatcagattgaatatgttgatcgtcgtaacaacgtgatgaaactgagccagggtgaatttgttgcaattgcccatattgaagcagttctgaccaccccaccgattcagcagctgtatgtttatggtaatagcgcacgtccgtatctgctggccgttgttgttccgacaccggaactgcgtgaacgtcatgcagatgataatgaactgcgtcgtgaagttctgacagcactgcgtagccatggtgaacgtaatggtctggcagcagttgaaattccgcgtgatgttattgttgaacgtaccccgtttagcctggaaaatggtctgctgacaggtattcgtaaactggcacgtccgcagctgaaagaacgttatggtgcacgtctggaagcactgtatgccgaactggccgatagccgtattacacgtctgcgtgatgtgaaagcagttgcagcccagcgtagcaccgttaccaccgttattgatgttgttaccgcaattctggatctggcggatggtgaagttaccgcagcagcacattttacagatctgggtggtgatagcctgaccgcagttaccgttggtaacgaactgcgcgatatttttgatgccgaagttccggttggtgtgctgaccagcccgagcagtaccctggcagatattgcggaacatattgatggccgtcatagcgaagcacgtccgaccgcagaaagcgttcatggcaccggtacaaccctgcgtgcagccgatctgaccctggataaatttctggatgaagaaacactgcgtgccgcaagtgatgttaccagtgcagccaccgatgttcgtaccgtgtttattaccggtgcaaccggttttctgggtcgctacctgacactggattggctgcgtcgtatggcaaaagttggtggtacagttatttgtctggtgcgtggtgccgatgatgacgcagcccgtgcgcgtctggatgcagcatttgatagcagcgatctgtggtctgaatatcagcgtctggcaaaagatcatctgcgcgtgctggcaggcgataaagatagcgatcatctggcactgacaccggatgtgtgggatgaactggcaaaaagcgttgatctgattattgatccggcagcactggttaatcatgtactgccgtatcgcgaactgtttggtccgaatgttagcggcaccgcagaactgatccgtctggcagttaccaccacccgtaaaccgtatgtgtatatttcaaccgtgggtgttggtgatcaggttgctccgggtagctttaccgaagatcctgatattcgtgaaatgagcagcgtgcgtgaaatcaatgatacctatgcaaatggttacggcaatagcaaatgggcaggcgaagttctgctggcacaggcacatgaacgttttgaactgccggttagcgtttttcgttgtgatatgattgttgcggatgatcataccattggtcagctgaatctgccggatatgtttactcgcctgctgatgagcgttctggcaacaggtctggcaccgcgtagcttttatcagctggcgaccgatggtagtgcacaagaggcacattttgatgcgctgccggtggatttcctggccgaagcaattaatacactgtgggttaaagatggtgcccgtacctttaatgcaatgaatccgcatgccgatggtattggttttgatcagtatattcgttggctgattgatagcggtgaacaaattagcctggtggataattatgatgattggtatcgtcgctttggtgccgcactggcggatctgcctgaaaaacagcgtcgtggtagcctgattccgctgctgcacaattatgttcatccgatgacaccgcataatcgtggtatggcaagcgcagatcgttttcatgatgcagttcgtacagcaggcgttggtcagagcagcgatattccgcatattacccctcagattattgaaaattatgcacgtagcctgcgtggcctgggtgtgatttaaaggaggacatacaatggtcgatatgaaaactacgcatacctccctcccctttgccggacatacgctgcattttgttgagttcgatccggcgaatttttgtgagcaggatttactctggctgccgcactacgcacaactgcaacacgctggacgtaaacgtaaaacagagcatttagccggacggatcgctgctgtttatgctttgcgggaatatggctataaatgtgtgcccgcaatcggcgagctacgccaacctgtctggcctgcggaggtatacggcagtattagccactgtgggactacggcattagccgtggtatctcgtcaaccgattggcattgatatagaagaaattttttctgtacaaaccgcaagagaattgacagacaacattattacaccagcggaacacgagcgactcgcagactgcggtttagccttttctctggcgctgacactggcattttccgccaaagagagcgcatttaaggcaagtgagatccaaactgatgcaggttttctggactatcagataattagctggaataaacagcaggtcatcattcatcgtgagaatgagatgtttgctgtgcactggcagataaaagaaaagatagtcataacgctgtgccaacacgattaattgacaacatctggtacgattcgcccgcagccatcactgaccacgggcgaaagtgtaaagcaggtgccttaccatcctgacctgacaaccggatatgcgggatccccgggtaccg

SEQ ID NO: 100 - DNA, 3387 bp, Gordonia effusa
atgagcgatcagccgaatgcactgccgagcgcaattgaaccgctgaatccggatccgcaggcaaccgagcagattagccattgtgcaaccattgcagaactggttcgtgttctggcagaaagctatggtgatcgtccggcactgggttggcgtaataatagcgatccgagcagctggcatagcatgacctatcgtgatctggccgaacgtgcagatagcatggcacgtctgctgcatagcaccctgggtgttgcagaaaatgatcgtgttgcaaccgttggttttaccagcgcagaatataccattgcaagcctggcagttggtacactgggtgcaatggaagttccgctgcagaatgcaggtagcgttgatgtttgggcagcaattctgaccgaaaccgattgtgttagcgcagttgttgcagcagatcagctgccgagcattgcccgtctggcggaaagcggcacctataccggtctgcgtcatgttctggtttttgatattggtagccgtgatggcaccaccctggatgatgcagcacgtcgtctggttgccgcaggcacccaggttcatctgcgtcagcctggtgcagaaccgaccacccctccggcaccgctgccgcagattaccgcaaacccggatcgtgtggcactgctgatttataccagcggtagcacaggtgcaccgaaaggtgcaatgtataccgaaacagcagttacccgtctgtttcagagcggtctgagtggtctgggtcgtgcaaccgatggtcatggttggattaccctgaactttatgccgatgagccatgttatgggtcgtagtaccctgtggcagaccctgggtaatggtggcaccgcatattttacaccgcgtgcagatctggctgaactgctgaccgatctggcagccgttcagccgacggatctgcagtttgttccgcgtatttgggatatgctgtatcaagaatatgttcgtctgacagatcaggatgttagcgaacaggatgcactgacccgtatgcgtgaacattatttcggcacccgtaccgcaaccgcaattaccggtagcgcaccgattagtgatgaagttcgtcgttttgttgaagcaatgctgccggttccgctgattgaaggttatggtagcaccgaagcagccggtgttagcattgatggtcgtattcagcgtccgcctgttgttgattataaactgctggatgtgccggaactgggttatctgagcaccgatcgtccgcatccgcgtggtgagctgctggttaaaaccgatcatatttttgccggttattacaatcgtccggatctgaccagcagcgtttttgatgatcagggttattatcgtaccggtgatattgttgccgaaaccggtccggatcagattgaatatgttgatcgtcgtaacaacgtgatgaaactgagccagggtgaatttgttgcaattgcccatattgaagcagttctgaccaccccaccgattcagcagctgtatgtttatggtaatagcgcacgtccgtatctgctggccgttgttgttccgacaccggaactgcgtgaacgtcatgcagatgataatgaactgcgtcgtgaagttctgacagcactgcgtagccatggtgaacgtaatggtctggcagcagttgaaattccgcgtgatgttattgttgaacgtaccccgtttagcctggaaaatggtctgctgacaggtattcgtaaactggcacgtccgcagctgaaagaacgttatggtgcacgtctggaagcactgtatgccgaactggccgatagccgtattacacgtctgcgtgatgtgaaagcagttgcagcccagcgtagcaccgttaccaccgttattgatgttgttaccgcaattctggatctggcggatggtgaagttaccgcagcagcacattttacagatctgggtggtgatagcctgaccgcagttaccgttggtaacgaactgcgcgatatttttgatgccgaagttccggttggtgtgctgaccagcccgagcagtaccctggcagatattgcggaacatattgatggccgtcatagcgaagcacgtccgaccgcagaaagcgttcatggcaccggtacaaccctgcgtgcagccgatctgaccctggataaatttctggatgaagaaacactgcgtgccgcaagtgatgttaccagtgcagccaccgatgttcgtaccgtgtttattaccggtgcaaccggttttctgggtcgctacctgacactggattggctgcgtcgtatggcaaaagttggtggtacagttatttgtctggtgcgtggtgccgatgatgacgcagcccgtgcgcgtctggatgcagcatttgatagcagcgatctgtggtctgaatatcagcgtctggcaaaagatcatctgcgcgtgctggcaggcgataaagatagcgatcatctggcactgacaccggatgtgtgggatgaactggcaaaaagcgttgatctgattattgatccggcagcactggttaatcatgtactgccgtatcgcgaactgtttggtccgaatgttagcggcaccgcagaactgatccgtctggcagttaccaccacccgtaaaccgtatgtgtatatttcaaccgtgggtgttggtgatcaggttgctccgggtagctttaccgaagatcctgatattcgtgaaatgagcagcgtgcgtgaaatcaatgatacctatgcaaatggttacggcaatagcaaatgggcaggcgaagttctgctggcacaggcacatgaacgttttgaactgccggttagcgtttttcgttgtgatatgattgttgcggatgatcataccattggtcagctgaatctgccggatatgtttactcgcctgctgatgagcgttctggcaacaggtctggcaccgcgtagcttttatcagctggcgaccgatggtagtgcacaagaggcacattttgatgcgctgccggtggatttcctggccgaagcaattaatacactgtgggttaaagatggtgcccgtacctttaatgcaatgaatccgcatgccgatggtattggttttgatcagtatattcgttggctgattgatagcggtgaacaaattagcctggtggataattatgatgattggtatcgtcgctttggtgccgcactggcggatctgcctgaaaaacagcgtcgtggtagcctgattccgctgctgcacaattatgttcatccgatgacaccgcataatcgtggtatggcaagcgcagatcgttttcatgatgcagttcgtacagcaggcgttggtcagagcagcgatattccgcatattacccctcagattattgaaaattatgcacgtagcctgcgtggcctgggtgtgatttaa

SEQ ID NO: 101 - DNA, 819 bp, Escherichia coli
atggaaacctatgctgtttttggtaatccgatagcccacagcaaatcgccattcattcatcagcaatttgctcagcaactgaatattgaacatccctatgggcgcgtgttggcacccatcaatgatttcatcaacacactgaacgctttctttagtgctggtggtaaaggtgcgaatgtgacggtgccttttaaagaagaggcttttgccagagcggatgagcttactgaacgggcagcgttggctggtgctgttaataccctcatgcggttagaagatggacgcctgctgggtgacaataccgatggtgtaggcttgttaagcgatctggaacgtctgtcttttatccgccctggtttacgtattctgcttatcggcgctggtggagcatctcgcggcgtactactgccactcctttccctggactgtgcggtgacaataactaatcggacggtatcccgcgcggaagagttggctaaattgtttgcgcacactggcagtattcaggcgttgagtatggacgaactggaaggtcatgagtttgatctcattattaatgcaacatccagtggcatcagtggtgatattccggcgatcccgtcatcgctcattcatccaggcatttattgctatgacatgttctatcagaaaggaaaaactccttttctggcatggtgtgagcagcgaggctcaaagcgtaatgctgatggtttaggaatgctggtggcacaggcggctcatgcctttcttctctggcacggtgttctgcctgacgtagaaccagttataaagcaattgcaggaggaattgtccgcgtga

SEQ ID NO: 102 - protein, 272 aa, Escherichia coli
METYAVFGNPIAHSKSPFIHQQFAQQLNIEHPYGRVLAPINDFINTLNAFFSAGGKGANVTVPFKEEAFARADELTERAALAGAVNTLMRLEDGRLLGDNTDGVGLLSDLERLSFIRPGLRILLIGAGGASRGVLLPLLSLDCAVTITNRTVSRAEELAKLFAHTGSIQALSMDELEGHEFDLIINATSSGISGDIPAIPSSLIHPGIYCYDMFYQKGKTPFLAWCEQRGSKRNADGLGMLVAQAAHAFLLWHGVLPDVEPVIKQLQEELSA